European Patent Specification EP 3 247 724 B1, published March 12, 2025. Title: Therapeutic Molecules. Applicant: Crescendo Biologics Limited. The sequence listing filed with the application follows.

SEQUENCE LISTING (466 sequences)

SEQ ID NO: 1 - protein, 5 aa, Artificial Sequence
  clone
SYSMY

SEQ ID NO: 2 - protein, 17 aa, Artificial Sequence
  clone
NIKQDGSEKYYVDSVKG

SEQ ID NO: 3 - protein, 10 aa, Artificial Sequence
  clone
GEILPLHFDY

SEQ ID NO: 4 - protein, 119 aa, Artificial Sequence
  clone
EVQLVESGGGLVQPGGSLRLSCAASGFTFSSYSMYWVRQAPGKGLEWVANIKQDGSEKYYVDSVKGRFTISRDNAKNSLFLQMNSLRAEDTAVYYCAKGEILPLHFDYWGQGTLVTVSS

SEQ ID NO: 5 - protein, 5 aa, Artificial Sequence
  clone
SYSMY

SEQ ID NO: 6 - protein, 17 aa, Artificial Sequence
  clone
EIKQDGSVQYYVSDVKG

SEQ ID NO: 7 - protein, 10 aa, Artificial Sequence
  clone
GEILPLYFDY

SEQ ID NO: 8 - protein, 119 aa, Artificial Sequence
  clone
EVQLVESGGGLVQPGGSLRLSCAASGFTFSSYSMYWVRQAPGKGLEWVAEIKQDGSVQYYVSDVKGRFTISRDNAKNSLYLQMNSLRAEDTAVYYCAKGEILPLYFDYWGQGTLVTVSS

SEQ ID NO: 9 - protein, 5 aa, Artificial Sequence
  clone
SYSMY

SEQ ID NO: 10 - protein, 17 aa, Artificial Sequence
  clone
EIKQDGSVQYYVDSVKG

SEQ ID NO: 11 - protein, 10 aa, Artificial Sequence
  clone
GEILPLYFDY

SEQ ID NO: 12 - protein, 119 aa, Artificial Sequence
  clone
EVQLVESGGGLVQPGGSLRLSCAASGFTFSSYSMYWVRQAPGKGLEWVAEIKQDGSVQYYVDSVKGRFTISRDNAKNSLYLQMNSLRAEDTAVYYCAKGEILPLYFDYWGQGTLVTVSS

SEQ ID NO: 13 - protein, 5 aa, Artificial Sequence
  clone
SYSMY

SEQ ID NO: 14 - protein, 17 aa, Artificial Sequence
  clone
EIKQTGSVQYYVDSVKG

SEQ ID NO: 15 - protein, 10 aa, Artificial Sequence
  clone
GEILPLYFDY

SEQ ID NO: 16 - protein, 119 aa, Artificial Sequence
  clone
EVQLVESGGGLVQPGGSLRLSCAASGFTFSSYSMYWVRQAPGKGLEWVAEIKQTGSVQYYVDSVKGRFTISRDNAKNSLYLQMNSLRAEDTAVYYCAKGEILPLYFDYWGQGTLVTVSS

SEQ ID NO: 17 - protein, 5 aa, Artificial Sequence
  clone
SYSMY

SEQ ID NO: 18 - protein, 17 aa, Artificial Sequence
  clone
EIKPTGSVQYYVDSVKG

SEQ ID NO: 19 - protein, 10 aa, Artificial Sequence
  clone
GEILPLYFDY

SEQ ID NO: 20 - protein, 119 aa, Artificial Sequence
  clone
EVQLVESGGGLVQPGGSLRLSCAASGFTFSSYSMYWVRQAPGKGLEWVAEIKPTGSVQYYVDSVKGRFTISRDNAKNSLYLQMNSLRAEDTAVYYCAKGEILPLYFDYWGQGTLVTVSS

SEQ ID NO: 21 - protein, 5 aa, Artificial Sequence
  clone
SYSMY

SEQ ID NO: 22 - protein, 17 aa, Artificial Sequence
  clone
EIKQDGSEQYYVDSVKG

SEQ ID NO: 23 - protein, 10 aa, Artificial Sequence
  clone
GEILPLYFDY

SEQ ID NO: 24 - protein, 119 aa, Artificial Sequence
  clone
EVQLVESGGGLVQPGGSLRLSCAASGFTFSSYSMYWVRQAPGKGLEWVAEIKQDGSEQYYVDSVKGRFTISRDNAKNSLYLQMNSLRAEDTAVYYCAKGEILPLYFDYWGQGTLVTVSS

SEQ ID NO: 25 - protein, 5 aa, Artificial Sequence
  clone
SYGMY

SEQ ID NO: 26 - protein, 17 aa, Artificial Sequence
  clone
KIEQDGSEEYYVDSVKG

SEQ ID NO: 27 - protein, 10 aa, Artificial Sequence
  clone
GEILPLYFDY

SEQ ID NO: 28 - protein, 119 aa, Artificial Sequence
  clone
QVQLVESGGGLVQPGGSLRLSCAASGFTFSSYGMYWVRQAPGKGLEWVAKIEQDGSEEYYVDSVKGRFTISRDNAKKSLYLQMNSLRAEDTAVYYCAKGEILPLYFDYWGQGTLVTVSS

SEQ ID NO: 29 - protein, 5 aa, Artificial Sequence
  clone
SYGMY

SEQ ID NO: 30 - protein, 17 aa, Artificial Sequence
  clone
KIEQDGSEKYYVDSVKG

SEQ ID NO: 31 - protein, 10 aa, Artificial Sequence
  clone
GEILPLYFDY

SEQ ID NO: 32 - protein, 119 aa, Artificial Sequence
  clone
QVQLVESGGGLVQPGGSLRLSCAASGFTFSSYGMYWVRQAPGKGLEWVAKIEQDGSEKYYVDSVKGRFTISRDNAKNSLFLQMNSLRAEDTAVYYCAKGEILPLYFDYWGQGTLVTVSS

SEQ ID NO: 33 - protein, 5 aa, Artificial Sequence
  clone
SYGMY

SEQ ID NO: 34 - protein, 17 aa, Artificial Sequence
  clone
EIKQDGSEKYYVDSVKG

SEQ ID NO: 35 - protein, 10 aa, Artificial Sequence
  clone
GEILPLYFDY

SEQ ID NO: 36 - protein, 119 aa, Artificial Sequence
  clone
QVQLVESGGGLVQPGGSLRLSCAASGFTFSSYGMYWVRQAPGKGLEWVAEIKQDGSEKYYVDSVKGRFTISRDNAKNSLYLQMNSLRAEDTAVYYCAKGEILPLYFDYWGQGTLVTVSS

SEQ ID NO: 37 - protein, 5 aa, Artificial Sequence
  clone
SYRMY

SEQ ID NO: 38 - protein, 17 aa, Artificial Sequence
  clone
SIEQDGSEEYYVDSVKG

SEQ ID NO: 39 - protein, 10 aa, Artificial Sequence
  clone
GEILPLYFDY

SEQ ID NO: 40 - protein, 119 aa, Artificial Sequence
  clone
EVQLVESGGGLVQPGGSLRLSCAASGFTFSSYRMYWVRQAPGKGLEWVASIEQDGSEEYYVDSVKGRFTISRDNAKKSLFLQMNSLRAEDTAVYYCAKGEILPLYFDYWGQGTLVTVSS

SEQ ID NO: 41 - protein, 5 aa, Artificial Sequence
  clone
SYQMY

SEQ ID NO: 42 - protein, 17 aa, Artificial Sequence
  clone
SIKQDGSEEYYVDSVKG

SEQ ID NO: 43 - protein, 10 aa, Artificial Sequence
  clone
GEILPLYFDY

SEQ ID NO: 44 - protein, 119 aa, Artificial Sequence
  clone
EVQLVESGGGLVQPGGSLRLSCAASGFTFSSYQMYWVRQAPGKGLEWVASIKQDGSEEYYVDSVKGRFTISRDNAKNSLFLQMNSLRAEDTAVYYCAKGEILPLYFDYWGQGTLVTVSS

SEQ ID NO: 45 - protein, 5 aa, Artificial Sequence
  clone
SYGMY

SEQ ID NO: 46 - protein, 17 aa, Artificial Sequence
  clone
KIEQDGSEEYYVDSVKG

SEQ ID NO: 47 - protein, 10 aa, Artificial Sequence
  clone
GEILPLYFDY

SEQ ID NO: 48 - protein, 10 aa, Artificial Sequence
  clone
GEILPLYFDY

SEQ ID NO: 49 - protein, 5 aa, Artificial Sequence
  clone
SYGMY

SEQ ID NO: 50 - protein, 17 aa, Artificial Sequence
  clone
SIEQDGSEKYYVDSVKG

SEQ ID NO: 51 - protein, 10 aa, Artificial Sequence
  clone
GEILPLYFDY

SEQ ID NO: 52 - protein, 119 aa, Artificial Sequence
  clone
EVQLVESGGGLVQPGGSLRLSCAASGFTFSSYGMYWVRQAPGKGLEWVASIEQDGSEKYYVDSVKGRFTISRDNAKNSLYLQMNSLRAEDTAVYYCAKGEILPLYFDYWGQGTLVTVSS

SEQ ID NO: 53 - protein, 5 aa, Artificial Sequence
  clone
SYRMY

SEQ ID NO: 54 - protein, 17 aa, Artificial Sequence
  clone
SIEQDGSEEYYVDSVKG

SEQ ID NO: 55 - protein, 10 aa, Artificial Sequence
  clone
GEILPLYFDY

SEQ ID NO: 56 - protein, 119 aa, Artificial Sequence
  clone
EVQLVESGGGLVQRGGSLRLSCAASGFTFSSYRMYWVRQAPGKGLEWVASIEQDGSEEYYVDSVKGRFTISRDNAKKSLFLQMNSLRAEDTAVYYCAKGEILPLYFDYWGQGTLVTVSS

SEQ ID NO: 57 - protein, 5 aa, Artificial Sequence
  clone
SYSMY

SEQ ID NO: 58 - protein, 17 aa, Artificial Sequence
  clone
EIRQDGSEQYYVDSVKG

SEQ ID NO: 59 - protein, 10 aa, Artificial Sequence
  clone
GEILPLYFDY

SEQ ID NO: 60 - protein, 119 aa, Artificial Sequence
  clone
EVQLVESGGGLVQPGGSLRLSCAASGFTFSSYSMYWVRQAPGKGLEWVAEIRQDGSEQYYVDSVKGRFTISRDNAKNSLYLQMNSLRAEDTAVYYCAKGEILPLYFDYWGQGTLVTVSS

SEQ ID NO: 61 - protein, 5 aa, Artificial Sequence
  clone
SYSMY

SEQ ID NO: 62 - protein, 17 aa, Artificial Sequence
  clone
EIKQDGSEQYYVDSVKG

SEQ ID NO: 63 - protein, 10 aa, Artificial Sequence
  clone
GEILPLYFDY

SEQ ID NO: 64 - protein, 119 aa, Artificial Sequence
  clone
EVQLVESGGGLVQPGGSLRLSCAASGFTFSSYSMYWVRQAPGKGLEWVAEIKQDGSEQYYVDSVKGRFTISRDNAKNSLYLQMNGLRAEDTAVYYCAKGEILPLYFDYWGQGTLVTVSS

SEQ ID NO: 65 - protein, 5 aa, Artificial Sequence
  clone
SYSMY

SEQ ID NO: 66 - protein, 17 aa, Artificial Sequence
  clone
EIKPTGSVQYYVSDVKG

SEQ ID NO: 67 - protein, 10 aa, Artificial Sequence
  clone
GEILPLYFDY

SEQ ID NO: 68 - protein, 119 aa, Artificial Sequence
  clone
EVQLVESGGGLVQPGGSLRLSCAASGFTFSSYSMYWVRQAPGKGLEWVAEIKPTGSVQYYVSDVKGRFTISRDNAKNSLYLQMNSLRAEDTAVYYCAKGEILPLYFDYWGQGTLVTVSS

SEQ ID NO: 69 - protein, 5 aa, Artificial Sequence
  clone
SYSMY

SEQ ID NO: 70 - protein, 17 aa, Artificial Sequence
  clone
EIKQDGSVQYYVGGVKG

SEQ ID NO: 71 - protein, 10 aa, Artificial Sequence
  clone
GEILPLYFDY

SEQ ID NO: 72 - protein, 119 aa, Artificial Sequence
  clone
EVQLVESGGGLVQPGGSLRLSCAASGFTFSSYSMYWVRQAPGKGLEWVAEIKQDGSVQYYVGGVKGRFTISRDNAKNSLYLQMNSLRAEDTAVYYCAKGEILPLYFDYWGQGTLVTVSS

SEQ ID NO: 73 - protein, 5 aa, Artificial Sequence
  clone
SYGMY

SEQ ID NO: 74 - protein, 17 aa, Artificial Sequence
  clone
EIKQDGSEKYYVDSVKG

SEQ ID NO: 75 - protein, 10 aa, Artificial Sequence
  clone
GEILPLYFDY

SEQ ID NO: 76 - protein, 119 aa, Artificial Sequence
  clone
EVQLVESGGGLVQPGGSLRLSCATSGFTFSSYGMYWVRQAPGKGLEWVAEIKQDGSEKYYVDSVKGRFTISRDNAKNSLYLQMNSLRAEDTAVYYCAKGEILPLYFDYWGQGTLVTVSS

SEQ ID NO: 77 - protein, 5 aa, Artificial Sequence
  clone
SYGMY

SEQ ID NO: 78 - protein, 17 aa, Artificial Sequence
  clone
KIEQDGSEEYYADSVKG

SEQ ID NO: 79 - protein, 10 aa, Artificial Sequence
  clone
GEILPLYFDY

SEQ ID NO: 80 - protein, 119 aa, Artificial Sequence
  clone
EVQLVESGGGLVQPGGSLRLSCAASGFTFSSYGMYWVRQAPGKGLEWVAKIEQDGSEEYYADSVKGRFTISRDNAKKSLYLQMNSLRAEDTAVYYCAKGEILPLYFDYWGQGTLVTVSS

SEQ ID NO: 81 - protein, 5 aa, Artificial Sequence
  clone
SYSMY

SEQ ID NO: 82 - protein, 17 aa, Artificial Sequence
  clone
EIKQDGSEQYYVDSVKG

SEQ ID NO: 83 - protein, 10 aa, Artificial Sequence
  clone
GEILPLYFDY

SEQ ID NO: 84 - protein, 119 aa, Artificial Sequence
  clone
EVQLVESGGGLVLPGGSLRLSCAASGFTFSSYSMYWVRQAPGKGLEWVAEIKQDGSEQYYVDSVKGRFTISRDNAKNSLYLQMNSLRAEDTAVYYCAKGEILPLYFDYWGQGTLVTVSS

SEQ ID NO: 85 - protein, 5 aa, Artificial Sequence
  clone
SYGMY

SEQ ID NO: 86 - protein, 17 aa, Artificial Sequence
  clone
KIEQDGSEEYYVDSVKG

SEQ ID NO: 87 - protein, 10 aa, Artificial Sequence
  clone
GEILPLYFDY

SEQ ID NO: 88 - protein, 119 aa, Artificial Sequence
  clone
EVQLVESGGGLVRPGGSLRLSCAASGFTFSSYGMYWVRQAPGKGLEWVAKIEQDGSEEYYVDSVKGRFTISRDNAKKSLYLQMNSLRAEDTAVYYCAKGEILPLYFDYWGQGTLVTVSS

SEQ ID NO: 89 - protein, 5 aa, Artificial Sequence
  clone
SYGMY

SEQ ID NO: 90 - protein, 17 aa, Artificial Sequence
  clone
EIKQDGSEKYYVDSVKG

SEQ ID NO: 91 - protein, 10 aa, Artificial Sequence
  clone
GEILPLYFDY

SEQ ID NO: 92 - protein, 119 aa, Artificial Sequence
  clone
QVQLVESGGGLVQPGGSLRLSCAASGFTFSSYGMYWVRQAPGKGLEWVAEIKQDGSEKYYVDSVKGRFTISRDNAKNSLFLQMNSLRAEDTAVYYCAKGEILPLYFDYWGQGTLVTVSS

SEQ ID NO: 93 - protein, 5 aa, Artificial Sequence
  clone
SYGMY

SEQ ID NO: 94 - protein, 17 aa, Artificial Sequence
  clone
EIKQDGSEQYYVDSVKG

SEQ ID NO: 95 - protein, 10 aa, Artificial Sequence
  clone
GEILPLYFDY

SEQ ID NO: 96 - protein, 119 aa, Artificial Sequence
  clone
QVQLVESGGGLVQPGGSLRLSCAASGFTFSSYGMYWVRQAPGKGLEWVAEIKQDGSEQYYVDSVKGRFTISRDNAKNSLFLQMNSLRAEDTAVYYCAKGEILPLYFDYWGQGTLVTVSS

SEQ ID NO: 97 - protein, 5 aa, Artificial Sequence
  clone
SYEMY

SEQ ID NO: 98 - protein, 17 aa, Artificial Sequence
  clone
SIKQDGSEQYYVDSVKG

SEQ ID NO: 99 - protein, 10 aa, Artificial Sequence
  clone
GEILPLYFDY

SEQ ID NO: 100 - protein, 119 aa, Artificial Sequence
  clone
EVQLVESGGGLVQPGGSLRLSCAASGFTFSSYEMYWVRQAPGKGLEWVASIKQDGSEQYYVDSVKGRFTISRDNAKNSLYLQMNSLRAEDTAVYYCAKGEILPLYFDYWGQGTLVTVSS

SEQ ID NO: 101 - protein, 5 aa, Artificial Sequence
  clone
SYGMY

SEQ ID NO: 102 - protein, 17 aa, Artificial Sequence
  clone
RIGQDGSEEYYVDSVKG

SEQ ID NO: 103 - protein, 10 aa, Artificial Sequence
  clone
GEILPLYFDY

SEQ ID NO: 104 - protein, 119 aa, Artificial Sequence
  clone
QVQLVESGGGLVQPGGSLRLSCAASGFTFSSYGMYWVRQAPGKGLEWVARIGQDGSEEYYVDSVKGRFTISRDNAKNSLYLQMNSLRAEDTAVYYCAKGEILPLYFDYWGQGTLVTVSS

SEQ ID NO: 105 - protein, 5 aa, Artificial Sequence
  clone
SYRMY

SEQ ID NO: 106 - protein, 17 aa, Artificial Sequence
  clone
SIEQDGSEEYYVDSVKG

SEQ ID NO: 107 - protein, 10 aa, Artificial Sequence
  clone
GEILPLYFDY

SEQ ID NO: 108 - protein, 119 aa, Artificial Sequence
  clone
EVQLVESGGGLVQPGGSLRLSCAASGFTFSSYRMYWVRQAPGKGLEWVASIEQDGSEEYYVDSVKGRFTISRDNAKKSLFLQMNSLRAGDTAVYYCAKGEILPLYFDYWGQGTLVTVSS

SEQ ID NO: 109 - protein, 5 aa, Artificial Sequence
  clone
SYRMY

SEQ ID NO: 110 - protein, 17 aa, Artificial Sequence
  clone
SIEQDGSEEYYVDSVKG

SEQ ID NO: 111 - protein, 10 aa, Artificial Sequence
  clone
GEILPLYFDY

SEQ ID NO: 112 - protein, 119 aa, Artificial Sequence
  clone
EVQLVESGGGLVQPGGSLRLSCAASGFTFSSYRMYWVRQAPGKGLEWVASIEQDGSEEYYVDSVKGRFTISRDNAKKSLFLQMNSLRAEDTAVYYCAKGEILPLYFDYWGQGTLVAVSS

SEQ ID NO: 113 - protein, 5 aa, Artificial Sequence
  clone
SYSMY

SEQ ID NO: 114 - protein, 17 aa, Artificial Sequence
  clone
SIDQDGSEEYYVDSVKG

SEQ ID NO: 115 - protein, 10 aa, Artificial Sequence
  clone
GEILPLYFDY

SEQ ID NO: 116 - protein, 119 aa, Artificial Sequence
  clone
EVQLVESGGGLVQPGGSLRLSCAASGFTFSSYSMYWVRQAPGKGLEWVASIDQDGSEEYYVDSVKGRFTISRDNAKKSLYLQMNSLRAEDTAVYYCAKGEILPLYFDYWGQGTLVTVSS

SEQ ID NO: 117 - protein, 5 aa, Artificial Sequence
  clone
SYRMY

SEQ ID NO: 118 - protein, 17 aa, Artificial Sequence
  clone
SIDQDGSEEYYVDSVKG

SEQ ID NO: 119 - protein, 10 aa, Artificial Sequence
  clone
GEILPLYFDY

SEQ ID NO: 120 - protein, 119 aa, Artificial Sequence
  clone
EVQLVESGGGLVQPGGSLRLSCAASGFTFSSYRMYWVRQAPGKGLEWVASIDQDGSEEYYVDSVKGRFTISRDNAKNSLYLQMNSLRAEDTAVYYCAKGEILPLYFDYWGQGTLVTVSS

SEQ ID NO: 121 - protein, 5 aa, Artificial Sequence
  clone
SYNMY

SEQ ID NO: 122 - protein, 5 aa, Artificial Sequence
  clone
SYNMY

SEQ ID NO: 123 - protein, 10 aa, Artificial Sequence
  clone
GEILPLYFDY

SEQ ID NO: 124 - protein, 119 aa, Artificial Sequence
  clone
QVQLVESGGGLVQPGGSLRLSCAASGFTFSSYNMYWVRQAPGKGLEWVANIEQDGSEEYYVDSVKGRFTISRDNAKNSLYLQMNSLRAEDTAVYYCAKGEILPLYFDYWGQGTLVTVSS

SEQ ID NO: 125 - protein, 5 aa, Artificial Sequence
  clone
SYRMY

SEQ ID NO: 126 - protein, 17 aa, Artificial Sequence
  clone
GIEQDGSEEYYVDSVKG

SEQ ID NO: 127 - protein, 10 aa, Artificial Sequence
  clone
GEILPLYFDY

SEQ ID NO: 128 - protein, 119 aa, Artificial Sequence
  clone
QVQLVESGGGLVQPGGSLRLSCAASGFTFSSYRMYWVRQAPGKGLEWVAGIEQDGSEEYYVDSVKGRFTISRDNAKNSLYLQMNSLRAEDTAVYYCAKGEILPLYFDYWGQGTLVTVSS

SEQ ID NO: 129 - protein, 5 aa, Artificial Sequence
  clone
SYGMY

SEQ ID NO: 130 - protein, 17 aa, Artificial Sequence
  clone
GIEQDGSEKYYVDSVKG

SEQ ID NO: 131 - protein, 10 aa, Artificial Sequence
  clone
GEILPLYFDY

SEQ ID NO: 132 - protein, 119 aa, Artificial Sequence
  clone
EVQLVESGGGLVQPGGSLRLSCAASGFTFSSYGMYWVRQAPGKGLEWVAGIEQDGSEKYYVDSVKGRFTISRDNAKNSLYLQMNSLRAEDTAVYYCAKGEILPLYFDYWGQGTLVTVSS

SEQ ID NO: 133 - protein, 5 aa, Artificial Sequence
  clone
SYGMY

SEQ ID NO: 134 - protein, 17 aa, Artificial Sequence
  clone
GIEQDGSEKYYVDSVKG

SEQ ID NO: 135 - protein, 10 aa, Artificial Sequence
  clone
GEILPLYFDY

SEQ ID NO: 136 - protein, 119 aa, Artificial Sequence; identical to SEQ ID NO: 132
  clone

SEQ ID NO: 137 - protein, 5 aa, Artificial Sequence
  clone
SYGMY

SEQ ID NO: 138 - protein, 17 aa, Artificial Sequence
  clone
GIEQDGSEKYYVDSVKG

SEQ ID NO: 139 - protein, 10 aa, Artificial Sequence
  clone
GEILPLYFDY

SEQ ID NO: 140 - protein, 119 aa, Artificial Sequence
  clone
EVQLVESGGGLVQPGGSLRLSCAASGFTFSSYGMYWVRQAPGKGLEWVAGIEQDGSEKYYVDSVKGRFTISRDNAKKSLYLQMNSLRAEDTAVYYCAKGEILPLYFDYWGQGTLVTVSS

SEQ ID NO: 141 - protein, 5 aa, Artificial Sequence
  clone
SYGMY

SEQ ID NO: 142 - protein, 17 aa, Artificial Sequence
  clone
GIEQDGSEEYYVDSVKG

SEQ ID NO: 143 - protein, 10 aa, Artificial Sequence
  clone
GEILPLYFDY

SEQ ID NO: 144 - protein, 119 aa, Artificial Sequence
  clone
EVQLVESGGGLVQPGGSLRLSCAASGFTFSSYGMYWVRQAPGKGLEWVAGIEQDGSEEYYVDSVKGRFTISRDNAKNSLFLQMNSLRAEDTAVYYCAKGEILPLYFDYWGQGTLVTVSS

SEQ ID NO: 145 - protein, 5 aa, Artificial Sequence
  clone
SYGMY

SEQ ID NO: 146 - protein, 17 aa, Artificial Sequence
  clone
RIEQDGSEQYYVDSVKG

SEQ ID NO: 147 - protein, 10 aa, Artificial Sequence
  clone
GEILPLYFDY

SEQ ID NO: 148 - protein, 119 aa, Artificial Sequence
  clone
EVQLVESGGGLVQPGGSLRLSCAASGFTFSSYGMYWVRQAPGKGLEWVARIEQDGSEQYYVDSVKGRFTISRDNAKNSLYLQMNSLRAEDTAVYYCAKGEILPLYFDYWGQGTLVTVSS

SEQ ID NO: 149 - protein, 5 aa, Artificial Sequence
  clone
SYGMY

SEQ ID NO: 150 - protein, 17 aa, Artificial Sequence
  clone
NIKQDGSEEYYVDSVKG

SEQ ID NO: 151 - protein, 10 aa, Artificial Sequence
  clone
GEILPLYFDY

SEQ ID NO: 152 - protein, 119 aa, Artificial Sequence
  clone
EVQLVESGGGLVQPGGSLRLSCAASGFTFSSYGMYWVRQAPGKGLEWVANIKQDGSEEYYVDSVKGRFTISRDNAKNSLYLQMNSLRAEDTAVYYCAKGEILPLYFDYWGQGTLVTVSS

SEQ ID NO: 153 - protein, 5 aa, Artificial Sequence
  clone
SYGMY

SEQ ID NO: 154 - protein, 17 aa, Artificial Sequence
  clone
NIKQDGSEEYYVDSVKG

SEQ ID NO: 155 - protein, 10 aa, Artificial Sequence
  clone
GEILPLYFDY

SEQ ID NO: 156 - protein, 119 aa, Artificial Sequence; identical to SEQ ID NO: 152
  clone

SEQ ID NO: 157 - protein, 5 aa, Artificial Sequence
  clone
SYGMY

SEQ ID NO: 158 - protein, 17 aa, Artificial Sequence
  clone
NIEQDGSEKYYVDSVKG

SEQ ID NO: 159 - protein, 10 aa, Artificial Sequence
  clone
GEILPLHFDY

SEQ ID NO: 160 - protein, 119 aa, Artificial Sequence
  clone
EVQLVESGGGLVQPGGSLRLSCAASGFMFSSYGMYWVRQAPGKGLEWVANIEQDGSEKYYVDSVKGRFTISRDNAKKSLYLQMNSLRAEDTAVYYCAKGEILPLHFDYWGQGTLVTVSS

SEQ ID NO: 161 - protein, 5 aa, Artificial Sequence
  clone
SYGMY

SEQ ID NO: 162 - protein, 17 aa, Artificial Sequence
  clone
NIEQDGSEKYYVDSVKG

SEQ ID NO: 163 - protein, 10 aa, Artificial Sequence
  clone
GEILPLHFDY

SEQ ID NO: 164 - protein, 119 aa, Artificial Sequence
  clone
EVQLVESGGGLVKPGGSLRLSCAASGFMFSSYGMYWVRQAPGKGLEWVANIEQDGSEKYYVDSVKGRFTISRDNAKKSLYLQMNSLRAEDTAVYYCAKGEILPLHFDYWGQGTLVTVSS

SEQ ID NO: 165 - protein, 5 aa, Artificial Sequence
  clone
SYGMY

SEQ ID NO: 166 - protein, 17 aa, Artificial Sequence
  clone
NIKQDGSEQYYVDSVKG

SEQ ID NO: 167 - protein, 10 aa, Artificial Sequence
  clone
GEILPLHFDY

SEQ ID NO: 168 - protein, 119 aa, Artificial Sequence
  clone
EVQLVESGGGLVQPGGSLRLSCAASGFTFSSYGMYWVRQAPGKGLEWVANIKQDGSEQYYVDSVKGRFTISRDNAKKSLYLQMNSLRAEDTAVYYCAKGEILPLHFDYWGQGTLVTVSS

SEQ ID NO: 169 - protein, 5 aa, Artificial Sequence
  clone
SYSMY

SEQ ID NO: 170 - protein, 17 aa, Artificial Sequence
  clone
NIKQDGSEKYYVDSVKG

SEQ ID NO: 171 - protein, 10 aa, Artificial Sequence
  clone
GEILPLHFDY

SEQ ID NO: 172 - protein, 119 aa, Artificial Sequence
  clone
EVQLVESGGGLVQPGGSLRLSCAVSGFTFSSYSMYWVRQAPGKGLEWVANIKQDGSEKYYVDSVKGRFTISRDNAKNSLYLQMNSLRAEDTAVYYCAKGEILPLHFDYWGQGTLVTVSS

SEQ ID NO: 173 - protein, 5 aa, Artificial Sequence
  clone
SYSMY

SEQ ID NO: 174 - protein, 17 aa, Artificial Sequence
  clone
NIKQDGSEKYYVDSVKG

SEQ ID NO: 175 - protein, 10 aa, Artificial Sequence
  clone
GEILPLYFDH

SEQ ID NO: 176 - protein, 119 aa, Artificial Sequence
  clone
EVQLVESGGGLVQPGGSLRLSCAASGFTFSSYSMYWVRQAPGKGLEWVANIKQDGSEKYYVDSVKGRFTISRDNAKNSLYLQMNSLRAEDTAVYYCAKGEILPLYFDHWGQGTLVTVSS

SEQ ID NO: 177 - protein, 5 aa, Artificial Sequence
  clone
SYWMY

SEQ ID NO: 178 - protein, 17 aa, Artificial Sequence
  clone
KIKQDGSEKYYVDSVKG

SEQ ID NO: 179 - protein, 10 aa, Artificial Sequence
  clone
GEILPLQFDY

SEQ ID NO: 180 - protein, 119 aa, Artificial Sequence
  clone
EVQLVESGGGLVQRGGSLRLSCAASGFTFSSYWMYWVRQAPGKGLEWVAKIKQDGSEKYYVDSVKGRFTISRDNAKNSLFLQMNSLRAEDTAVYYCAKGEILPLQFDYWGQGTLVTVSS

SEQ ID NO: 181 - protein, 5 aa, Artificial Sequence
  clone
SYWMY

SEQ ID NO: 182 - protein, 17 aa, Artificial Sequence
  clone
KINQDGSEKYYVDSVKG

SEQ ID NO: 183 - protein, 10 aa, Artificial Sequence
  clone
GEILPLQFDY

SEQ ID NO: 184 - protein, 119 aa, Artificial Sequence
  clone
EVQLVESGGGLVQRGGSLRLSCAASGFTFSSYWMYWVRQAPGKGLEWVAKINQDGSEKYYVDSVKGRFTISRDNAKNSLYLQMNSLRAEDTAVYYCAKGEILPLQFDYWGQGTLVTVSS

SEQ ID NO: 185 - protein, 5 aa, Artificial Sequence
  clone
SYWMY

SEQ ID NO: 186 - protein, 17 aa, Artificial Sequence
  clone
KINQDGSEKYYVDSVKG

SEQ ID NO: 187 - protein, 10 aa, Artificial Sequence
  clone
GEILPLQFDY

SEQ ID NO: 188 - protein, 119 aa, Artificial Sequence
  clone
QVQLVESGGGLVQRGGSLRLSCAASGFTFSSYWMYWVRQAPGKGLEWVAKINQDGSEKYYVDSVKGRFTISRDNAKNSLYLQMNSLRAEDTAVYYCAKGEILPLQFDYWGQGTLVTVSS

SEQ ID NO: 189 - protein, 5 aa, Artificial Sequence
  clone
SYWMY

SEQ ID NO: 190 - protein, 17 aa, Artificial Sequence
  clone
KINQDGSEKYYVDSVKG

SEQ ID NO: 191 - protein, 10 aa, Artificial Sequence
  clone
GEILPLQFDY

SEQ ID NO: 192 - protein, 119 aa, Artificial Sequence
  clone
QVQLVESGGGLVQPGGSLRLSCAASGFTFSSYWMYWVRQAPGKGLEWVAKINQDGSEKYYVDSVKGRFTISRDNAKNSLYLQMNSLRAEDTAVYYCAKGEILPLQFDYWGQGTLVTVSP

SEQ ID NO: 193 - protein, 5 aa, Artificial Sequence
  clone
SYQMY

SEQ ID NO: 194 - protein, 17 aa, Artificial Sequence
  clone
EIKQDGSEQYYVDSVKG

SEQ ID NO: 195 - protein, 10 aa, Artificial Sequence
  clone
GEILPLYFDH

SEQ ID NO: 196 - protein, 119 aa, Artificial Sequence
  clone
EVQLVESGGGLVQPGGSLRLSCAASGFTFSSYQMYWVRQAPGKGLEWVAEIKQDGSEQYYVDSVKGRFTISRDNAKNSLFLQMNSLRAEDTAVYYCAKGEILPLYFDHWGQGTLVTVSS

SEQ ID NO: 197 - protein, 5 aa, Artificial Sequence
  clone
SYSMI

SEQ ID NO: 198 - protein, 17 aa, Artificial Sequence
  clone
DIKQDGSEKYYVDSVKG

SEQ ID NO: 199 - protein, 10 aa, Artificial Sequence
  clone
GEVLPLYFDY

SEQ ID NO: 200 - protein, 119 aa, Artificial Sequence
  clone
EVQLVESGGGLVQPGGSLRLSCAASGFTFSSYSMIWVRQAPGKGLEWVADIKQDGSEKYYVDSVKGRFTISRDNAKNSLYLQMNSLRAEDTAVYYCAKGEVLPLYFDYWGQGTLVTVSS

SEQ ID NO: 201 - protein, 5 aa, Artificial Sequence
  clone
SYSMI

SEQ ID NO: 202 - protein, 17 aa, Artificial Sequence
  clone
DIKQDGSEKYYVDSVKG

SEQ ID NO: 203 - protein, 10 aa, Artificial Sequence
  clone
GEVLPLYFDY

SEQ ID NO: 204 - protein, 119 aa, Artificial Sequence; identical to SEQ ID NO: 200
  clone

SEQ ID NO: 205 - protein, 5 aa, Artificial Sequence
  clone
SYNMY

SEQ ID NO: 206 - protein, 17 aa, Artificial Sequence
  clone
EIDQDGSEKYYVDSVKG

SEQ ID NO: 207 - protein, 10 aa, Artificial Sequence
  clone
GEILPLYFDH

SEQ ID NO: 208 - protein, 119 aa, Artificial Sequence
  clone
EVQLVESGGGLVQPGGSLRLSCAASGFTFSSYNMYWVRQAPGKGLEWVAEIDQDGSEKYYVDSVKGRFTISRDNAKNSLFLQMNSLRAEDTAVYYCAKGEILPLYFDHWGQGTLVTVSS

SEQ ID NO: 209 - protein, 5 aa, Artificial Sequence
  clone
SYRMY

SEQ ID NO: 210 - protein, 17 aa, Artificial Sequence
  clone
SIEQDGSEEYYVDSVKG

SEQ ID NO: 211 - protein, 10 aa, Artificial Sequence
  clone
GEILPLYFDY

SEQ ID NO: 212 - protein, 119 aa, Artificial Sequence
  clone
QVQLVESGGGLVQPGGSLRLSCAASGFTFSSYRMYWVRQAPGKGLEWVASIEQDGSEEYYVDSVKGRFTISRDNAKRSLFLQMSSLRAEDSAVYYCAKGEILPLYFDYWGQGTLVTVSS

SEQ ID NO: 213 - protein, 5 aa, Artificial Sequence
  clone
SYQMY

SEQ ID NO: 214 - protein, 17 aa, Artificial Sequence
  clone
GIEQDGSEEYYVDSVKG

SEQ ID NO: 215 - protein, 10 aa, Artificial Sequence
  clone
GEILPLYFDH

SEQ ID NO: 216 - protein, 119 aa, Artificial Sequence
  clone
QVQLVESGGGLVQPGGSLRLSCAASGFTFSSYQMYWVRQAPGKGLEWVAGIEQDGSEEYYVDSVKGRFTISRDNAKNSLYLQMNSLRAEDTAVYYCAKGEILPLYFDHWGQGTLVTVSS

SEQ ID NO: 217 - protein, 5 aa, Artificial Sequence
  clone
SYEMY

SEQ ID NO: 218 - protein, 17 aa, Artificial Sequence
  clone
NIKQDGSEKYYVDSVKG

SEQ ID NO: 219 - protein, 17 aa, Artificial Sequence
  clone
NIKQDGSEKYYVDSVKG

SEQ ID NO: 220 - protein, 119 aa, Artificial Sequence
  clone
QVQLVESGGGLVQPGGSLRLSCAVSGFTFSSYEMYWVRQAPGKGLEWVANIKQDGSEKYYVDSVKGRFTISRDNAKNSLYLQMNSLRAEDTAMYYCAKGEILPLHFDYRGQGTLVTVSS

SEQ ID NO: 221 - protein, 5 aa, Artificial Sequence
  clone
SYSMY

SEQ ID NO: 222 - protein, 17 aa, Artificial Sequence
  clone
NIKQDGSEKYYVDSVKG

SEQ ID NO: 223 - protein, 10 aa, Artificial Sequence
  clone
GEILPLYFDY

SEQ ID NO: 224 - protein, 119 aa, Artificial Sequence
  clone
EVQLVESGGGLVQPGGSLRLSCAVSGFTFSSYSMYWVRQAPGKGLEWVANIKQDGSEKYYVDSVKGRFTISRDNAKNLLYLQMNSLRVEDTAVYYCAKGEILPLYFDYRGQGTLVTVSS

SEQ ID NO: 225 - protein, 5 aa, Artificial Sequence
  clone
SYRMY

SEQ ID NO: 226 - protein, 17 aa, Artificial Sequence
  clone
SINQDGSEKYYVDSVKG

SEQ ID NO: 227 - protein, 10 aa, Artificial Sequence
  clone
GEILPLHFDY

SEQ ID NO: 228 - protein, 119 aa, Artificial Sequence
  clone
QVQLVESGGGLVQPGGSLRLSCAVSGFTFSSYRMYWVRQAPGKGLEWVASINQDGSEKYYVDSVKGRFTISRDNAKNSLYLQMNSLRAEDTAMYYCAKGEILPLHFDYRGQGTLVTVSS

SEQ ID NO: 229 - protein, 5 aa, Artificial Sequence
  clone
SYRMY

SEQ ID NO: 230 - protein, 17 aa, Artificial Sequence
  clone
SINQDGSEKYYVDSVKG

SEQ ID NO: 231 - protein, 17 aa, Artificial Sequence
  clone
SINQDGSEKYYVDSVKG

SEQ ID NO: 232 - protein, 119 aa, Artificial Sequence
  clone
QVQLVESGGGMVQPGGSLRLSCAVSGFTFSSYRMYWVRQAPGKGLEWVASINQDGSEKYYVDSVKGRFTISRDNAKNSLYLQMNSLRAEDTAMYYCAKGEILPLHFDYRGQGTLVTVSS

SEQ ID NO: 233 - protein, 5 aa, Artificial Sequence
  clone
SYWMY

SEQ ID NO: 234 - protein, 17 aa, Artificial Sequence
  clone
KIKQDGTEKYYVDSVKG

SEQ ID NO: 235 - protein, 10 aa, Artificial Sequence
  clone
GEILPHYFDY

SEQ ID NO: 236 - protein, 119 aa, Artificial Sequence
  clone
QVQLQESGGDWVQPGGSLRLSCGASGFTFSSYWMYWVRQAPGKGLEWVAKIKQDGTEKYYVDSVKGRFTISRDNAKNSLYLQMNSLRAEDTAVYYCAKGEILPHYFDYWGQGTLVTVSS

SEQ ID NO: 237 - protein, 5 aa, Artificial Sequence
  clone
NYSMY

SEQ ID NO: 238 - protein, 17 aa, Artificial Sequence
  clone
NIKQDGSEEYYVDSVKG

SEQ ID NO: 239 - protein, 10 aa, Artificial Sequence
  clone
GEILPLYFDH

SEQ ID NO: 240 - protein, 119 aa, Artificial Sequence
  clone
EVQLVESGGGLVQPGGSLRLSCTASGFTFSNYSMYWVRQAPGKGLEWVANIKQDGSEEYYVDSVKGRFTISRDNARNSLYLQMISLRAEDTAVYYCAKGEILPLYFDHWGQGTLVTVSS

SEQ ID NO: 241 - protein, 5 aa, Artificial Sequence
  clone
NYSMY

SEQ ID NO: 242 - protein, 17 aa, Artificial Sequence
  clone
NIKQDGSEEYYVDSVKG

SEQ ID NO: 243 - protein, 10 aa, Artificial Sequence
  clone
GEILPLYFDH

SEQ ID NO: 244 - protein, 119 aa, Artificial Sequence; identical to SEQ ID NO: 240
  clone

SEQ ID NO: 245 - protein, 5 aa, Artificial Sequence
  clone
NYSMY

SEQ ID NO: 246 - protein, 17 aa, Artificial Sequence
  clone
NIKQDGSEEYYVDSVKG

SEQ ID NO: 247 - protein, 10 aa, Artificial Sequence
  clone
GEILPLYFDH

SEQ ID NO: 248 - protein, 119 aa, Artificial Sequence
  clone
QVQLVESGGGLVQPGGSLRLSCTASGFTFSNYSMYWVRQAPGKGLEWVANIKQDGSEEYYVDSVKGRFTISRDNARNSLYLQMISLRAEDTAVYYCAKGEILPLYFDHWGQGTLVTVSS

SEQ ID NO: 249 - protein, 5 aa, Artificial Sequence
  clone
SYGMG

SEQ ID NO: 250 - protein, 17 aa, Artificial Sequence
  clone
KIKQDGSEKDYVDSVKG

SEQ ID NO: 251 - protein, 17 aa, Artificial Sequence
  clone
KIKQDGSEKDYVDSVKG

SEQ ID NO: 252 - protein, 118 aa, Artificial Sequence
  clone
QVQLVESGGGLVQPGGSLRLSCAASGFTFSSYGMGWVRQAPGKGLEWVAKIKQDGSEKDYVDSVKGRFTISRDNAKKSLFLQMNSLRAEDTAVYYCARESIFGIPEDWGQGTLVTVSS

SEQ ID NO: 253 - protein, 5 aa, Artificial Sequence
  clone
AYWMG

SEQ ID NO: 254 - protein, 17 aa, Artificial Sequence
  clone
KIKQDGSEKDYVDSVKG

SEQ ID NO: 255 - protein, 9 aa, Artificial Sequence
  clone
ESIFGIPED

SEQ ID NO: 256 - protein, 118 aa, Artificial Sequence
  clone
EVQLVESGGGLVQSGGSLRLSCAASGFTFSAYWMGWVRQAPGKGLEWVAKIKQDGSEKDYVDSVKGRFTISRDNAKNSLFLQMNSLRAEDTAVYYCARESIFGIPEDWGQGTLVTVSS

SEQ ID NO: 257 - protein, 5 aa, Artificial Sequence
  clone
AYWMG

SEQ ID NO: 258 - protein, 17 aa, Artificial Sequence
  clone
KIKQDGSEKDYVDSVKG

SEQ ID NO: 259 - protein, 9 aa, Artificial Sequence
  clone
ESIFGTPED

SEQ ID NO: 260 - protein, 118 aa, Artificial Sequence
  clone
QVQLVESGGGLVQPGGSLRLSCTTSGFTFSAYWMGWVRQAPGKGLEWVAKIKQDGSEKDYVDSVKGRFTISRDNAKKSLFLQMNSLRAEDTAVYYCARESIFGTPEDWGQGTLVTVSS

SEQ ID NO: 261 - protein, 5 aa, Artificial Sequence
  clone
SYWMS

SEQ ID NO: 262 - protein, 17 aa, Artificial Sequence
  clone
KIKQDGSEKDYVDSVKG

SEQ ID NO: 263 - protein, 9 aa, Artificial Sequence
  clone
ESIFGIPED

SEQ ID NO: 264 - protein, 118 aa, Artificial Sequence
  clone
QVQLVESGGGLVQPGGSLRLSCAASGFTFSSYWMSWVRQAPGKGLEWVAKIKQDGSEKDYVDSVKGRFTISRDNAKNSLFLQMNSLRAEDTAVYYCARESIFGIPEDWGQGTLVTVSS

SEQ ID NO: 265 - protein, 5 aa, Artificial Sequence
  clone
GYWMG

SEQ ID NO: 266 - protein, 17 aa, Artificial Sequence
  clone
KIKQDGSEKDYVDSVKG

SEQ ID NO: 267 - protein, 9 aa, Artificial Sequence
  clone
ESIFGIPED

SEQ ID NO: 268 - protein, 118 aa, Artificial Sequence
  clone
QVQLVESGGGLVQPGGSLRLSCAASGFTFSGYWMGWVRQAPGKGLEWVAKIKQDGSEKDYVDSVKGRFTISRDNAKNSLFLQMNSLRAEDTAVYYCARESIFGIPEDWGQGTLVTVSS

SEQ ID NO: 269 - protein, 5 aa, Artificial Sequence
  clone
AYWMG

SEQ ID NO: 270 - protein, 17 aa, Artificial Sequence
  clone
KIKQDGSEKDYVDSVKG

SEQ ID NO: 271 - protein, 9 aa, Artificial Sequence
  clone
ESIFGTPED

SEQ ID NO: 272 - protein, 118 aa, Artificial Sequence
  clone
EVQLVESGGGLVQPGGSLRLSCAASGFTFSAYWMGWVRQAPGKGLEWVAKIKQDGSEKDYVDSVKGRFTISRDNAKKALFLQMNSLRAEDTAVYYCARESIFGTPEDWGQGTLVTVSS

SEQ ID NO: 273 - protein, 5 aa, Artificial Sequence
  clone
SYWMS

SEQ ID NO: 274 - protein, 17 aa, Artificial Sequence
  clone
NIKQDGSEKDYVDSVKG

SEQ ID NO: 275 - protein, 17 aa, Artificial Sequence
  clone
NIKQDGSEKDYVDSVKG

SEQ ID NO: 276 - protein, 118 aa, Artificial Sequence
  clone
EVQLVESGGGLVQPGGSLRLSCAASGFTFSSYWMSWVRQAPGKGLEWVANIKQDGSEKDYVDSVKGRFTISRDNAKNSLFLQMNSLRAEDTAVYYCARESIFGTPEDWGQGTLVTVSS

SEQ ID NO: 277 - protein, 5 aa, Artificial Sequence
  clone
GYWMG

SEQ ID NO: 278 - protein, 17 aa, Artificial Sequence
  clone
KIKQDGSEKDYVDSVKG

SEQ ID NO: 279 - protein, 9 aa, Artificial Sequence
  clone
ESIFGIPED

SEQ ID NO: 280 - protein, 118 aa, Artificial Sequence
  clone
EVQLVESGGGLVQPGGSLRLSCAASGFTFSGYWMGWVRQAPGKGLEWVAKIKQDGSEKDYVDSVKGRFTISRDNAKNSLFLQMNSLRAEDTAVYYCARESIFGIPEDWGQGTLVTVSS

SEQ ID NO: 281 - protein, 5 aa, Artificial Sequence
  clone
AYWMG

SEQ ID NO: 282 - protein, 17 aa, Artificial Sequence
  clone
KIKQDGSEKDYVDSVKG

SEQ ID NO: 283 - protein, 9 aa, Artificial Sequence
  clone
ESIFGIPED

SEQ ID NO: 284 - protein, 118 aa, Artificial Sequence
  clone
EVQLVESGGGLVQPGGSLRLSCAASGFTFSAYWMGWVRQAPGRGLEWVAKIKQDGSEKDYVDSVKGRFTISRDNAKNSLFLQMNSLRAEDTAVYYCARESIFGIPEDWGQGTLVTVSS

SEQ ID NO: 285 - protein, 5 aa, Artificial Sequence
  clone
GYYMH

SEQ ID NO: 286 - protein, 17 aa, Artificial Sequence
  clone
WINPNSGGTNYAQKFQG

SEQ ID NO: 287 - protein, 17 aa, Artificial Sequence
  clone
MDRDYYDTSGYFGWFDS

SEQ ID NO: 288 - protein, 126 aa, Artificial Sequence
  clone
QVQLVQSGAEVKKPGASVKVSCKASGYTFTGYYMHWVRQAPGQGLEWMGWINPNSGGTNYAQKFQGRVTMTRDTSISTAYMELSRLRSDDTAVYYCASMDRDYYDTSGYFGWFDSWGQGTLVTVSS

SEQ ID NO: 289 - protein, 5 aa, Artificial Sequence
  clone
AYYIN

SEQ ID NO: 290 - protein, 17 aa, Artificial Sequence
  clone
SIKPNTGATKYAQKFQG

SEQ ID NO: 291 - protein, 17 aa, Artificial Sequence
  clone
LDRDTWYPHSYAGWFDA

SEQ ID NO: 292 - protein, 126 aa, Artificial Sequence
  clone
QVQLVQSGAEVKKPGASVKVSCKASGYNADAYYINWVRQAPGQGLEWMGSIKPNTGATKYAQKFQGRVTITRDTSISTAYMELSRLRSDDTAVYYCASLDRDTWYPHSYAGWFDAWGQGTLVTVSS

SEQ ID NO: 293 - protein, 5 aa, Artificial Sequence
  clone
DYYLH

SEQ ID NO: 294 - protein, 17 aa, Artificial Sequence
  clone
WINPNTGTTKYAREFEG

SEQ ID NO: 295 - protein, 17 aa, Artificial Sequence
  clone
MDRDYYDTSGYFGWFDS

SEQ ID NO: 296 - protein, 126 aa, Artificial Sequence
  clone
QVQLVQSGAEVKKPGASVKVSCAASGYTFTDYYLHWVRQAPGQGLEWMGWINPNTGTTKYAREFEGRVTMTRDTSISTAYMELSRLRSDDTAVYYCASMDRDYYDTSGYFGWFDSWGQGTLVTVSS

SEQ ID NO: 297 - protein, 5 aa, Artificial Sequence
  clone
DYYLH

SEQ ID NO: 298 - protein, 17 aa, Artificial Sequence
  clone
WINPNTGTTKYAREFEG

SEQ ID NO: 299 - protein, 17 aa, Artificial Sequence
  clone
MDRDWRSPNDYFGWFDS

SEQ ID NO: 300 - protein, 126 aa, Artificial Sequence
  clone
QVQLVQSGAEVKKPGASVKVSCAASGYTFTDYYLHWVRQAPGQGLEWMGWINPNTGTTKYAREFEGRVTMTRDTSISTAYMELSRLRSDDTAVYYCASMDRDWRSPNDYFGWFDSWGQGTLVTVSS

SEQ ID NO: 301 - protein, 5 aa, Artificial Sequence
  clone
DYYLH

SEQ ID NO: 302 - protein, 17 aa, Artificial Sequence
  clone
WINPNTGTTKYAREFEG

SEQ ID NO: 303 - protein, 17 aa, Artificial Sequence
  clone
LDRDWRSPNDYFGWFDS

SEQ ID NO: 304 - protein, 126 aa, Artificial Sequence
  clone
QVQLVQSGAEVKKPGASVKVSCAASGYTFTDYYLHWVRQAPGQGLEWMGWINPNTGTTKYAREFEGRVTMTRDTSISTAYMELSRLRSDDTAVYYCASLDRDWRSPNDYFGWFDSWGQGTLVTVSS

SEQ ID NO: 305 - protein, 5 aa, Artificial Sequence
  clone
DYYLH

SEQ ID NO: 306 - protein, 17 aa, Artificial Sequence
  clone
WINPNTGTTKYAREFEG

SEQ ID NO: 307 - protein, 17 aa, Artificial Sequence
  clone
LDRDWRSPNDYYGWFDS

SEQ ID NO: 308 - protein, 126 aa, Artificial Sequence
  clone
QVQLVQSGAEVKKPGASVKVSCAASGYTFTDYYLHWVRQAPGQGLEWMGWINPNTGTTKYAREFEGRVTMTRDTSISTAYMELSRLRSDDTAVYYCASLDRDWRSPNDYYGWFDSWGQGTLVTVSS

SEQ ID NO: 309 - protein, 5 aa, Artificial Sequence
  clone
DYYLH

SEQ ID NO: 310 - protein, 17 aa, Artificial Sequence
  clone
WINPNTGTTKYAREFEG

SEQ ID NO: 311 - protein, 17 aa, Artificial Sequence
  clone
LDRDWRSPNDYYGWFDS

SEQ ID NO: 312 - protein, 126 aa, Artificial Sequence
  clone
QVQLVQSGAEVKKPGASVKVSCKASGYTFTDYYLHWVRQAPGQGLEWMGWINPNTGTTKYAREFEGRVTITRDTSISTAYMELSRLRSDDTAVYYCASLDRDWRSPNDYYGWFDSWGQGTLVTVSS

SEQ ID NO: 313 - protein, 5 aa, Artificial Sequence
  clone
DYYLH

SEQ ID NO: 314 - protein, 17 aa, Artificial Sequence
  clone
WINPNTGTTKYAREFEG

SEQ ID NO: 315 - protein, 17 aa, Artificial Sequence
  clone
LDRDWRSPNDYFGWFDS

SEQ ID NO: 316 - protein, 126 aa, Artificial Sequence
  clone
QVQLVQSGAEVKKPGASVKVSCAASGYTLTDYYLHWVRQAPGQGLEWMGWINPNTGTTKYAREFEGRVTMTRDTSISTAYMELSGLRSDDTAVYYCASLDRDWRSPNDYFGWFDSWGQGTLVTVSS

SEQ ID NO: 317 - protein, 5 aa, Artificial Sequence
  clone
AYHIN

SEQ ID NO: 318 - protein, 17 aa, Artificial Sequence
  clone
SIKPNSGATKYAQKFQG

SEQ ID NO: 319 - protein, 17 aa, Artificial Sequence
  clone
MDRDYYDTSGYFGWFDS

SEQ ID NO: 320 - protein, 126 aa, Artificial Sequence
  clone
QVQLVQSGAEVKKPGASVKVSCKASGYNFDAYHINWVRQAPGQGLEWMGSIKPNSGATKYAQKFQGRVTITRDTSISTAYMELSRLRSDDTAVYYCASMDRDYYDTSGYFGWFDSWGQGTLVTVSS

SEQ ID NO: 321 - protein, 5 aa, Artificial Sequence
  clone
AYHIN

SEQ ID NO: 322 - protein, 17 aa, Artificial Sequence
  clone
SIKPNSGATKYAQKFQG

SEQ ID NO: 323 - protein, 17 aa, Artificial Sequence
  clone
MDRDQFYFGDYFGWFDS

SEQ ID NO: 324 - protein, 126 aa, Artificial Sequence
  clone
QVQLVQSGAEVKKPGASVKVSCKASGYNFDAYHINWVRQAPGQGLEWMGSIKPNSGATKYAQKFQGRVTITRDTSISTAYMELSRLRSDDTAVYYCASMDRDQFYFGDYFGWFDSWGQGTLVTVSS

SEQ ID NO: 325 - protein, 5 aa, Artificial Sequence
  clone
AYHIN

SEQ ID NO: 326 - protein, 17 aa, Artificial Sequence
  clone
SIKPNSGATKYAQKFQG

SEQ ID NO: 327 - protein, 17 aa, Artificial Sequence
  clone
LDRDTWYPHSYFGWFDS

SEQ ID NO: 328 - protein, 126 aa, Artificial Sequence
  clone
QVQLVQSGAEVKKPGASVKVSCKASGYNFDAYHINWVRQAPGQGLEWMGSIKPNSGATKYAQKFQGRVTITRDTSISTAYMELSRLRSDDTAVYYCASLDRDTWYPHSYFGWFDSWGQGTLVTVSS

SEQ ID NO: 329 - protein, 5 aa, Artificial Sequence
  clone
AYHIN

SEQ ID NO: 330 - protein, 17 aa, Artificial Sequence
  clone
SIKPNSGATKYAQKFQG

SEQ ID NO: 331 - protein, 17 aa, Artificial Sequence
  clone
MDRDTWYPHSYFGWFDS

SEQ ID NO: 332 - protein, 126 aa, Artificial Sequence
  clone
QVQLVQSGAEVKKPGASVKVSCKASGYNFDAYHINWVRQAPGQGLEWMGSIKPNSGATKYAQKFQGRVTITRDTSISTAYMELSRLRSDDTAVYYCASMDRDTWYPHSYFGWFDSWGQGTLVTVSS

SEQ ID NO: 333 - protein, 5 aa, Artificial Sequence
  clone
AYHIN

SEQ ID NO: 334 - protein, 17 aa, Artificial Sequence
  clone
SIKPNSGATKYAQKFQG

SEQ ID NO: 335 - protein, 17 aa, Artificial Sequence
  clone
LDRDTWYPHSYAGWFDS

SEQ ID NO: 336 - protein, 126 aa, Artificial Sequence
  clone
QVQLVQSGAEVKKPGASVKVSCKASGYNFDAYHINWVRQAPGQGLEWMGSIKPNSGATKYAQKFQGRVTITRDTSISTAYMELSRLRSDDTAVYYCASLDRDTWYPHSYAGWFDSWGQGTLVTVSS

SEQ ID NO: 337 - protein, 5 aa, Artificial Sequence
  clone
AYYIN

SEQ ID NO: 338 - protein, 17 aa, Artificial Sequence
  clone
SIKPNSGATKYAQKFQG

SEQ ID NO: 339 - protein, 17 aa, Artificial Sequence
  clone
LDRDTWYPHSYFGWFDS

SEQ ID NO: 340 - protein, 126 aa, Artificial Sequence
  clone
QVQLVQSGAEVKKPGASVKVSCKASGYNSDAYYINWVRQAPGQGLEWMGSIKPNSGATKYAQKFQGRVTITRDTSISTAYMELSRLRSDDTAVYYCASLDRDTWYPHSYFGWFDSWGQGTLVTVSS

SEQ ID NO: 341 - protein, 5 aa, Artificial Sequence
  clone
SYWMN

SEQ ID NO: 342 - protein, 17 aa, Artificial Sequence
  clone
TIKQDGSEKYYVDSVKG

SEQ ID NO: 343 - protein, 11 aa, Artificial Sequence
  clone
GDTIFDGAFDI

SEQ ID NO: 344 - protein, 120 aa, Artificial Sequence
  clone
QVQLVESGGGLVQPGGSLRLSCAASGFTFSSYWMNWVRQAPGKGLEWVATIKQDGSEKYYVDSVKGRFTISRDNATNSLFLQMNSLRAEDTAVYYCARGDTIFDGAFDIWGQGTMVTVSS

SEQ ID NO: 345 - protein, 5 aa, Artificial Sequence
  clone
SYWMS

SEQ ID NO: 346 - protein, 17 aa, Artificial Sequence
  clone
NIKQDGSEKYYVDSVKG

SEQ ID NO: 347 - protein, 8 aa, Artificial Sequence
  clone
GQWPFFDY

SEQ ID NO: 348 - protein, 117 aa, Artificial Sequence
  clone
EVQLVESGGGLVQPGGSLRLSCAASGFTFSSYWMSWVRQAPGKGLEWVANIKQDGSEKYYVDSVKGRFTISRDNAKNSLYLQMNSLRAEDTAVYYCAHGQWPFFDYWGQGTMVTVSS

SEQ ID NO: 349 - DNA, 357 bp, Artificial Sequence
  VH 1.1
gaggtgcagctggtggagtctgggggaggcttggtccagcctggggggtccctgagactctcctgtgcagcctctggattcacctttagtagttattcgatgtactgggtccgccaggctccagggaaggggctggagtgggtggccaacataaagcaagatggaagtgagaaatactatgtggactctgtgaagggccgattcaccatctccagagacaacgccaagaactcactgtttctgcaaatgaatagcctgagagccgaggacacggctgtgtattactgtgcgaaaggggaaatactacccctccactttgactactggggccagggaaccctggtcactgtctcctca

SEQ ID NO: 350 - DNA, 357 bp, Artificial Sequence
  VH 1.2
gaggttcagttggtggaaagcggcggtggcctggtccagccgggtggtagcctgcgcctgtcctgcgcggctagcggtttcacgtttagcagctacagcatgtactgggtgcgtcaagcgccaggcaaaggtctggaatgggttgccgagattaagcaagacggttctgttcagtattatgtcagcgacgtgaagggtcgttttaccatcagccgtgacaacgcgaaaaacagcctgtatttgcagatgaattccctgcgcgctgaagataccgcggtgtattactgtgcgaaaggtgagattctgccgctgtacttcgattactggggccaaggcaccctggttactgtctcgagc

SEQ ID NO: 351 - DNA, 357 bp, Artificial Sequence
  VH 1.3
gaggtgcagctggtggagtctgggggaggcttggtccagcctggggggtccctgagactctcctgtgcagcctctggattcacctttagtagttatagcatgtactgggtccgccaggctccagggaaggggctggagtgggtggccgagataaagcaagatggaagtgtgcaatactatgtggactctgtgaagggccgattcaccatctccagagacaacgccaagaactcactgtatctgcaaatgaatagcctgagagccgaggacacggctgtgtattactgtgcgaaaggggaaatactacccctctactttgactactggggccagggaaccctggtcactgtctcttca

SEQ ID NO: 352 - DNA, 357 bp, Artificial Sequence
  VH 1.4
gaggttcagttggtggaaagcggcggtggcctggtccagccgggtggtagcctgcgcctgtcctgcgcggctagcggtttcacgtttagcagctacagcatgtactgggtgcgtcaagcgccaggcaaaggtctggaatgggttgccgagattaagcaaaccggttctgttcagtattatgtcgacagcgtgaagggtcgttttaccatcagccgtgacaacgcgaaaaacagcctgtatttgcagatgaattccctgcgcgctgaagataccgcggtgtattactgtgcgaaaggtgagattctgccgctgtacttcgattactggggccaaggcaccctggttactgtctcgagc

SEQ ID NO: 353 - DNA, 357 bp, Artificial Sequence
  VH 1.5
gaggttcagttggtggaaagcggcggtggcctggtccagccgggtggtagcctgcgcctgtcctgcgcggctagcggtttcacgtttagcagctacagcatgtactgggtgcgtcaagcgccaggcaaaggtctggaatgggttgccgagattaagccgaccggttctgttcagtattatgtcgacagcgtgaagggtcgttttaccatcagccgtgacaacgcgaaaaacagcctgtatttgcagatgaattccctgcgcgctgaagataccgcggtgtattactgtgcgaaaggtgagattctgccgctgtacttcgattactggggccaaggcaccctggttactgtctcgagc

SEQ ID NO: 354 - DNA, 357 bp, Artificial Sequence
  VH 1.6
gaggtgcagctggtggagtctgggggaggcttggtccagcctggggggtccctgagactctcctgtgcagcctctggattcacctttagtagttatagcatgtactgggtccgccaggctccagggaaggggctggagtgggtggccgagataaagcaagatggaagtgagcaatactatgtggactctgtgaagggccgattcaccatctccagagacaacgccaagaactcactgtatctgcaaatgaatagcctgagagccgaggacacggctgtgtattactgtgcgaaaggggaaatactacccctctactttgactactggggccagggaaccctggtcaccgtctcctca

SEQ ID NO: 355 - DNA, 357 bp, Artificial Sequence
  VH 1.7
caggtgcagctggtggagtctgggggaggcttggtccagcctggggggtccctgagactctcctgtgcagcctctggattcacctttagtagttatgggatgtactgggtccgccaggctccagggaaggggctggagtgggtggccaagatagagcaagatggaagtgaggaatactatgtggactctgtgaagggccgattcaccatctccagagacaacgccaagaagtcactgtatctgcaaatgaatagcctgagagccgaggacacggctgtgtattactgtgcgaaaggggaaatactacccctctactttgactactggggccagggaaccctggtcaccgtctcctca

SEQ ID NO: 356 - DNA, 357 bp, Artificial Sequence
  VH 1.8
caggtgcagctggtggagtctgggggaggcttggtccagcctggggggtccctgagactctcctgtgcagcctctggattcacctttagtagttatggtatgtactgggtccgccaggctccagggaaggggctggagtgggtggccaagatagagcaagatggaagtgagaaatactatgtggactctgtgaagggccgattcaccatctccagagacaacgccaagaactcactgtttctgcaaatgaatagcctgagagccgaggacacggctgtgtattactgtgcgaaaggggaaatactacccctctactttgactactggggccagggaaccctggtcaccgtctcctca

SEQ ID NO: 357 - DNA, 357 bp, Artificial Sequence
  VH 1.9
caggtgcagctggtggagtctgggggaggcttggtccagcctggggggtccctgagactctcctgtgcagcctctggattcacctttagtagttatggaatgtactgggtccgccaggctccagggaaggggctggagtgggtggccgagataaaacaagatggaagtgagaaatactatgtggactctgtgaagggccgattcaccatctccagagacaacgccaagaactcactgtatctgcaaatgaatagcctgagagccgaggacacggctgtgtattactgtgcgaaaggggaaatactacccctctactttgactactggggccagggaaccctggtcactgtctcttca

SEQ ID NO: 358 - DNA, 357 bp, Artificial Sequence
  VH 1.10
gaggtgcagctggtggagtctgggggaggcttggtccagcctggggggtccctgagactctcctgtgcagcctctggattcacctttagtagttatcgcatgtactgggtccgccaggctccagggaaggggctggagtgggtggccagcatagaacaagatggaagtgaggaatactatgtggactctgtgaagggccgattcaccatctccagagacaacgccaagaagtcactgtttctgcaaatgaatagcctgagagccgaggacacggctgtgtattactgtgcgaaaggggaaatactacccctctactttgactactggggccagggaaccctggtcactgtctcttca

SEQ ID NO: 359 - DNA, 357 bp, Artificial Sequence
  VH 1.11
gaggtgcagctggtggagtctgggggaggcttggtccagcctggggggtccctgagactctcctgtgcagcctctggattcacctttagtagttatcagatgtactgggtccgccaggctccagggaaggggctggagtgggtggccagcataaaacaagatggaagtgaggaatactatgtggactctgtgaagggccgattcaccatctccagagacaacgccaagaactcactgtttctgcaaatgaatagcctgagagccgaggacacggctgtgtattactgtgcgaaaggggaaatactacccctctactttgactactggggccagggaaccctggtcactgtctcttca

SEQ ID NO: 360 - DNA, 357 bp, Artificial Sequence
  VH 1.12
caggtgcagctggtggagtctgggggaggcttggtccagcctggggggtccctgagactctcctgtgcagcctctggattcacctttagtagttatgggatgtactgggtccgccaggctccagggaaggggctggagtgggtggccaagatagagcaagatggaagtgaggaatactatgtggactctgtgaagggccgattcaccatctccagagacaacgccaagaactcactgtatctgcaaatgaatagcctgagagccgaggacacggctgtgtattactgtgcgaaaggggaaatactacccctctactttgactactggggccagggaaccctggtcactgtctcctca

SEQ ID NO: 361 - DNA, 357 bp, Artificial Sequence
  VH 1.13
gaggtgcagctggtggagtctgggggaggcttggtccagcctggggggtccctgagactctcctgtgcagcctctggattcacctttagtagttatgggatgtactgggtccgccaggctccagggaaggggctggagtgggtggccagcatagaacaagatggaagtgagaaatactatgtggactctgtgaagggccgattcaccatctccagagacaacgccaagaactcactgtatctgcaaatgaatagcctgagagccgaggacacggctgtgtattactgtgcgaaaggggaaatactacccctctactttgactactggggccagggaaccctggtcaccgtctcctca

SEQ ID NO: 362 - DNA, 357 bp, Artificial Sequence
  VH 1.14
gaggtgcagctggtggagtctgggggaggcttggtccagcgtggggggtccctgagactctcctgtgcagcctctggattcacctttagtagttatcggatgtactgggtccgccaggctccagggaaggggctggagtgggtggccagcatagaacaagatggaagtgaggaatactatgtggactctgtgaagggccgattcaccatctccagagacaacgccaagaagtcactgtttctgcaaatgaatagcctgagagccgaggacacggctgtgtattactgtgcgaaaggggaaatactacccctctactttgactactggggccagggaaccctggtcactgtctcttca

SEQ ID NO: 363 - DNA, 357 bp, Artificial Sequence
  VH 1.15
gaggtgcagctggtggagtctgggggaggcttggtccagcctggggggtccctgagactctcctgtgcagcctctggattcacctttagtagttatagcatgtactgggtccgccaggctccagggaaggggctggagtgggtggccgagataaggcaagatggaagtgagcaatactatgtggactctgtgaagggccgattcaccatctccagagacaacgccaagaactcactgtatctgcaaatgaatagcctgagagccgaggacacggctgtgtattactgtgcgaaaggggaaatactacccctctactttgactactggggccagggaaccctggtcactgtctcttca

SEQ ID NO: 364 - DNA, 357 bp, Artificial Sequence
  VH 1.16
gaggtgcagctggtggagtctgggggaggcttggtccagcctggggggtccctgagactctcctgtgcagcctctggattcacctttagtagttatagcatgtactgggtccgccaggctccagggaaggggctggagtgggtggccgagataaagcaagatggaagtgagcaatactatgtggactctgtgaagggccgattcaccatctccagagacaacgccaagaactcactgtatctgcaaatgaatggcctgagagccgaggacacggctgtgtattactgtgcgaaaggggaaatactgcccctctacttcgactactggggccagggaaccctggtcactgtctcttca

SEQ ID NO: 365 - DNA, 357 bp, Artificial Sequence
  VH 1.17
gaggtgcagctggtggagtctgggggaggcttggtccagcctggggggtccctgagactctcctgtgcagcctctggattcacctttagtagttatagcatgtactgggtccgccaggctccagggaaggggctggagtgggtggccgagataaagccaaccgggagtgtgcaatactatgtgtccgacgtgaagggccgattcaccatctccagagacaacgccaagaactcactgtatctgcaaatgaatagcctgagagccgaggacacggctgtgtattactgtgcgaaaggggaaatactacccctctactttgactactggggccagggaaccctggtcactgtctcttca

SEQ ID NO: 366 - DNA, 357 bp, Artificial Sequence
  VH 1.18
gaggtgcagctggtggagtctgggggaggcttggtccagcctggggggtccctgagactctcctgtgcagcctctggattcacctttagtagttatagcatgtactgggtccgccaggctccagggaaggggctggagtgggtggccgagataaagcaagacggcagtgtgcaatactatgtggggggcgtgaagggccgattcaccatctccagagacaacgccaagaactcactgtatctgcaaatgaatagcctgagagccgaggacacggctgtgtattactgtgcgaaaggggaaatactacccctctactttgactactggggccagggaaccctggtcactgtctcttca

SEQ ID NO: 367 - DNA, 357 bp, Artificial Sequence
  VH 1.19
gaggtgcagctggtggagtctgggggaggcttggtccagcctggggggtccctgagactctcctgtgcaacctctggattcacctttagtagttatggaatgtactgggtccgccaggctccagggaaggggctggagtgggtggccgagataaaacaagatggaagtgagaaatactatgtggactccgtgaagggccgattcaccatctccagagacaacgccaagaactcactgtatctgcaaatgaatagcctgagagccgaggacacggctgtgtattactgtgcgaaaggggaaatactacccctctactttgactactggggccagggaaccctggtcactgtctcttca

SEQ ID NO: 368 - DNA, 357 bp, Artificial Sequence
  VH 1.20
gaggtgcagctggtggagtctgggggaggcctggtccagcctggggggtccctgagactctcctgtgcagcctctggattcacctttagtagttatgggatgtactgggtccgccaggctccagggaaggggctggagtgggtggccaagatagagcaagatggaagtgaggaatactatgcggactctgtgaagggccgattcaccatctccagagacaacgccaagaagtcactgtatctgcaaatgaatagcctgagagccgaggacacggctgtgtattactgtgcgaaaggggaaatactacccctctactttgactactggggccagggaaccctggtcactgtctcttca

SEQ ID NO: 369 - DNA, 357 bp, Artificial Sequence
  VH 1.21
gaggtgcagctggtggagtctgggggaggcttggtcctgcctggggggtccctgagactctcctgtgcggcctctggattcacctttagtagttatagcatgtactgggtccgccaggctccagggaaggggctggagtgggtggccgagataaagcaagatggaagtgagcaatactatgtggactctgtgaagggccgattcaccatctccagagacaacgccaagaactcactgtatctgcaaatgaatagcctgagagccgaggacacggctgtgtattactgtgcgaaaggggaaatactacccctctactttgactactggggccagggaaccctggtcactgtctcttca

SEQ ID NO: 370 - DNA, 357 bp, Artificial Sequence
  VH 1.22
gaggtgcagctggtggagtctgggggaggcttggtccggcctggggggtccctgagactctcctgtgcagcctctggattcacctttagtagttatgggatgtactgggtccgccaggctccagggaaggggctggagtgggtggccaagatagagcaagatggaagtgaggaatactatgtggactctgtgaagggccgattcaccatctccagagacaacgccaagaagtcactgtatctgcaaatgaatagcctgagagccgaggacacggccgtgtattactgtgcgaaaggggaaatactacccctctactttgactactggggccagggaaccctggtcactgtctcttca

SEQ ID NO: 371 - DNA, 354 bp, Artificial Sequence
  VH 2.1
caggtgcagctggtggagtctgggggaggcttggtccagcctggggggtccctgagactctcctgtgcagcctctggattcacctttagtagctatgggatgggctgggtccgccaggctccagggaaggggctggagtgggtggccaaaataaaacaagatggaagtgagaaagactatgtggactctgtgaagggccgattcaccatctccagagacaacgccaagaagtcactgtttctgcaaatgaacagcctgagagccgaggacacggctgtgtattattgtgcgagagagagtatatttggaatccccgaggactggggccagggaaccctggtcaccgtctcctca

SEQ ID NO: 372 - DNA, 378 bp, Artificial Sequence
  nucleic acid encoding VH 3.1
caggtgcagctggtgcagtctggggctgaggtgaagaagcctggggcctcagtgaaggtctcctgcaaggcttctggatacaccttcaccggctactatatgcactgggtgcgacaggcccctggacaagggcttgagtggatgggatggatcaaccctaacagtggtggcacaaactatgcacagaagtttcagggcagggtcaccatgaccagggacacgtccatcagcacagcctacatggagctgagcaggctgagatctgacgacacggccgtgtattactgtgcgagtatggatcgggattattatgatactagtggttactttggctggttcgactcctggggccagggaaccctggtcaccgtctcttca

SEQ ID NO: 373 - DNA, 378 bp, Artificial Sequence
  nucleic acid encoding VH 3.2
caggttcagctggtgcagtctggagctgaggtaaagaagcctggggcctcggtgaaggtctcctgtaaggcttccggatataacgcggacgcctattatataaattgggtgcgacaggcccctggacaaggtcttgagtggatgggaagtatcaagcctaataccggtgccacaaaatatgcacagaagtttcagggcagagtcaccataaccagggacacgtccatcagcacagcctacatggagctgagcaggctgagatctgacgacacggccgtgtattactgtgcgagtctggatcgggatacgtggtacccgcactcctacgcggggtggttcgacgcgtggggccagggaaccctggtcaccgtctcttca

SEQ ID NO: 374 - DNA, 378 bp, Artificial Sequence
  nucleic acid encoding VH 3.3
caggtgcagctggtgcagtctggggctgaggtgaagaagcctggggcctcagtgaaggtctcctgcgcagcttccggatacaccttcaccgactactatctgcactgggtgcgacaggcccctggacaagggcttgagtggatggggtggatcaaccctaacactggcaccacaaagtatgcacgggagtttgagggcagagtcaccatgaccagggacacgtccatcagcacagcctacatggagctgagcaggctgagatctgacgacacggccgtgtattactgtgcgagtatggatcgggattattatgatactagtggttactttggctggttcgactcctggggccagggaaccctggtcaccgtctcttca

SEQ ID NO: 375 - DNA, 378 bp, Artificial Sequence
  nucleic acid encoding VH 3.5
caggtccagctggtgcagtctggggctgaggtgaagaagcctggggcctcagtgaaggtctcctgcgcagcttccggatacaccttcaccgactactatctgcactgggtgcgacaggcccctggacaagggcttgagtggatggggtggatcaaccctaacactggcaccacaaagtatgcacgggagtttgagggcagagtcaccatgaccagggacacgtccatcagcacagcctacatggagctgagcaggctgagatctgacgacacggccgtgtattactgtgcgagtctggatcgggattggcgctcgcccaacgactactttggctggttcgactcgtggggccagggaaccctggtcaccgtctcttca

SEQ ID NO: 376 - DNA, 378 bp, Artificial Sequence
  nucleic acid encoding VH 3.6
caggtccagctggtgcagtctggggctgaggtgaagaagcctggggcctcagtgaaggtctcctgcgcagcttccggatacaccttcaccgactactatctgcactgggtgcgacaggcccctggacaagggcttgagtggatggggtggatcaaccctaacactggcaccacaaagtatgcacgggagtttgagggcagagtcaccatgaccagggacacgtccatcagcacagcctacatggagctgagcaggctgagatctgacgacacggccgtgtattactgtgcgagtctggatcgggattggcgctcgcccaacgactactacgggtggttcgactcgtggggccagggaaccctggtcaccgtctcttca

SEQ ID NO: 377 - DNA, 378 bp, Artificial Sequence
  nucleic acid encoding VH 3.9
caggtgcagctggtgcagtctggggctgaggtgaagaagcctggggcctcagtgaaggtctcctgtaaggcttccggatataacttcgacgcctatcatataaattgggtgcgacaggcccctggacaagggcttgagtggatgggaagtatcaagcctaatagtggtgccacaaaatatgcacagaagtttcagggcagagtcaccataaccagggacacgtccatcagcacagcctacatggagctgagcaggctgagatctgacgacacggccgtgtattactgtgcgagtatggatcgggattactatgatactagtggttactttggctggttcgactcctggggccagggaaccctggtcaccgtctcctca

SEQ ID NO: 378 - DNA, 378 bp, Artificial Sequence
  nucleic acid encoding VH 3.11
caggtgcagctggtgcagtctggggctgaggtgaagaagcctggggcctcagtgaaggtctcctgtaaggcttccggatataacttcgacgcctatcatataaattgggtgcgacaggcccctggacaaggtcttgagtggatgggaagtatcaagcctaatagtggtgccacaaaatatgcacagaagtttcagggcagagtcaccataaccagggacacgtccatcagcacagcctacatggagctgagcaggctgagatctgacgacacggccgtgtattactgtgcgagtctggatcgggatacgtggtacccgcactcctactttggctggttcgactcgtggggccagggaaccctggtcaccgtctcttca

SEQ ID NO: 379 - DNA, 378 bp, Artificial Sequence
  nucleic acid encoding VH 3.13
caggtccagctggtgcagtctggggctgaggtgaagaagcctggggcctcagtgaaggtctcctgtaaggcttccggatataacttcgacgcctatcatataaattgggtgcgacaggcccctggacaaggtcttgagtggatgggaagtatcaagcctaatagtggtgccacaaaatatgcacagaagtttcagggcagagtcaccataaccagggacacgtccatcagcacagcctacatggagctgagcaggctgagatctgacgacacggccgtgtattactgtgcgagtctggatcgggatacgtggtacccgcactcctacgcggggtggttcgactcgtggggccagggaaccctggtcaccgtctcttca

SEQ ID NO: 380 - DNA, 360 bp, Artificial Sequence
  nucleic acid encoding VH 4.1
caggtgcagctggtggagtctgggggaggcttggtccagcctggggggtccctgagactctcctgtgcagcctctggattcacctttagtagctattggatgaactgggtccgccaggctccagggaaggggctggaatgggtggccaccataaaacaagatggaagtgagaaatactatgtggactctgtgaagggccgattcaccatctccagagacaacgccacgaactcactgtttctgcaaatgaacagcctgagagccgaggacacggctgtgtattactgtgcgaggggagatacgattttcgacggtgcttttgatatctggggccaagggacaatggtcactgtctcctca

SEQ ID NO: 381 - DNA, 348 bp, Artificial Sequence
  nucleic acid encoding VH 5.1
gaggtgcagctggtggagtctgggggaggcttggtccagcctggggggtccctgagactctcctgtgcagcctctggattcacctttagtagctattggatgagctgggtccgccaggctccagggaaggggctggagtgggtggccaacataaagcaagatggaagtgagaaatactatgtggactctgtgaagggccgattcaccatctccagagacaacgccaagaactcactgtatctgcaaatgaacagcctgagagccgaggacacggctgtgtattactgtgcgcatcagtggcccttctttgactactggggccaagggacaatggtcactgtctcctca

SEQ ID NO: 382 - DNA, 73 bp, Artificial Sequence
  Primer
gccgctggattgttattactcgcggcccagccggccatggcccaggtbcagctggtgcagtctggggctgagg

SEQ ID NO: 383 - DNA, 65 bp, Artificial Sequence
  Primer
gccgctggattgttattactcgcggcccagccggccatggcccagatcaccttgaaggagtctgg

SEQ ID NO: 384 - DNA, 71 bp, Artificial Sequence
  Primer
gccgctggattgttattactcgcggcccagccggccatggccsaggtgcagctggtggagtctgggggagg

SEQ ID NO: 385 - DNA, 65 bp, Artificial Sequence
  Primer
gccgctggattgttattactcgcggcccagccggccatggcccaggtgcagctgcaggagtcggg

SEQ ID NO: 386 - DNA, 65 bp, Artificial Sequence
  Primer
gccgctggattgttattactcgcggcccagccggccatggcccaggtacagctgcagcagtcagg

SEQ ID NO: 387 - DNA, 54 bp, Artificial Sequence
  Primer
ccgtggtgatggtggtgatggctaccgccaccctcgagtgargagacrgtgacc

SEQ ID NO: 388 - DNA, 31 bp, Artificial Sequence
  primer
ctcgagggtggcggtagccatcaccaccatc

SEQ ID NO: 389 - DNA, 29 bp, Artificial Sequence
  primer
tccatggccatcgccggctgggccgcgag

SEQ ID NO: 390 - DNA, 34 bp, Artificial Sequence
  Primer
gctaccgccaccctcgagtgargagacrgtgacc

SEQ ID NO: 391 - DNA, 50 bp, Artificial Sequence
  Primer
ggaacagaccaccatggcccaggtbcagctggtgcagtctggggctgagg

SEQ ID NO: 392 - DNA, 23 bp, Artificial Sequence
  Primer
gacacggccgtgtattactgtgc

SEQ ID NO: 393 - DNA, 23 bp, Artificial Sequence
  Primer
gcacagtaatacacggccgtgtc

SEQ ID NO: 394 - protein, 98 aa, Artificial Sequence
  scaffold sequence
QVQLVQSGAEVKKPGASVKVSCKASGYTFTGYYMHWVRQAPGQGLEWMGWINPNSGGTNYAQKFQGRVTMTRDTSISTAYMELSRLRSDDTAVYYCAR

SEQ ID NO: 395 - DNA, 294 bp, Artificial Sequence
  scaffold sequence
caggtgcagctggtgcagtctggggctgaggtgaagaagcctggggcctcagtgaaggtctcctgcaaggcttctggatacaccttcaccggctactatatgcactgggtgcgacaggcccctggacaagggcttgagtggatgggatggatcaaccctaacagtggtggcacaaactatgcacagaagtttcagggcagggtcaccatgaccagggacacgtccatcagcacagcctacatggagctgagcaggctgagatctgacgacacggccgtgtattactgtgcgaga

SEQ ID NO: 396 - protein, 12 aa, Artificial Sequence
  C terminal extension
LEGGGSHHHHHH

SEQ ID NO: 397 - DNA, 71 bp, Artificial Sequence; identical to SEQ ID NO: 384
  primer

SEQ ID NO: 398 - DNA, 36 bp, Artificial Sequence
  primer
tggcggacccagtacatnybataactactaaaggtg

SEQ ID NO: 399 - DNA, 51 bp, Artificial Sequence
  primer
cacatagtattbctcacttccatcttgntytatsyyggccacccactccag

SEQ ID NO: 400 - DNA, 37 bp, Artificial Sequence
  primer
caagatggaagtgagvaatactatgtggactctgtga

SEQ ID NO: 401 - DNA, 45 bp, Artificial Sequence
  primer
aggctattcatttgcagawacagtgasttcttggcgttgtctctg

SEQ ID NO: 402 - DNA, 45 bp, Artificial Sequence
  primer
cagagacaacgccaagaastcactgtwtctgcaaatgaatagcct

SEQ ID NO: 403 - DNA, 36 bp, Artificial Sequence
  primer
agtatttcccctttcgcacagtaatacacagccgtg

SEQ ID NO: 404 - DNA, 67 bp, Artificial Sequence
  primer
cacggctgtgtattactgtgcgaaaggggaaatactacccctcyastttgacyactggggccaggga

SEQ ID NO: 405 - DNA, 54 bp, Artificial Sequence; identical to SEQ ID NO: 387
  primer

SEQ ID NO: 406 - DNA, 72 bp, Artificial Sequence
  Primer
gcactctcccctgttgaagctctttgtgacgggcgagctcaggccctgatgggtgacttcgcaggcgtagac

SEQ ID NO: 407 - DNA, 41 bp, Artificial Sequence
  Primer
gcagctaatacgactcactatagggagacagaccaccatgg

SEQ ID NO: 408 - DNA, 21 bp, Artificial Sequence
  Primer
gcactctcccctgttgaagct

SEQ ID NO: 409 - protein, 128 aa, Artificial Sequence
  clone
EVQLVESGGGLVQPGGSLRLSCAASGFTFSSYRMYWVRQAPGKGLEWVASIEQDGSEEYYVDSVKGRFTISRDNAKKSLFLQMNSLRAEDTAVYYCAKGEILPLYFDYWGQGTLVTVSSAAAHHHHHH

SEQ ID NO: 410 - protein, 128 aa, Artificial Sequence
  clone
EVQLVESGGGLVQPGGSLRLSCAASGFTFSSYSMYWVRQAPGKGLEWVAEIKQDGSVQYYVSDVKGRFTISRDNAKNSLYLQMNSLRAEDTAVYYCAKGEILPLYFDYWGQGTLVTVSSAAAHHHHHH

SEQ ID NO: 411 - protein, 120 aa, Artificial Sequence
  clone
EVQLVESGGGLVQPGGSLRLSCAASGFTFSSYSMYWVRQAPGKGLEWVAEIKQDGSVQYYVSDVKGRFTISRDNAKNSLYLQMNSLRAEDTAVYYCAKGEILPLYFDYWGQGTLVTVSSA

SEQ ID NO: 412 - protein, 128 aa, Artificial Sequence
  clone
EVQLVESGGGLVQPGGSLRLSCAASGFTFSSYSMYWVRQAPGKGLEWVAEIKQDGSVQYYVDSVKGRFTISRDNAKNSLYLQMNSLRAEDTAVYYCAKGEILPLYFDYWGQGTLVTVSSAAAHHHHHH

SEQ ID NO: 413 - protein, 120 aa, Artificial Sequence
  clone
EVQLVESGGGLVQPGGSLRLSCAASGFTFSSYSMYWVRQAPGKGLEWVAEIKQDGSVQYYVDSVKGRFTISRDNAKNSLYLQMNSLRAEDTAVYYCAKGEILPLYFDYWGQGTLVTVSSA

SEQ ID NO: 414 - protein, 131 aa, Artificial Sequence
  clone
EVQLVESGGGLVQPGGSLRLSCAASGFTFSSYSMYWVRQAPGKGLEWVAEIKQDGSEQYYVDSVKGRFTISRDNAKNSLYLQMNSLRAEDTAVYYCAKGEILPLYFDYWGQGTLVTVSSLEGGGSHHHHHH

SEQ ID NO: 415 - protein, 131 aa, Artificial Sequence
  clone
QVQLVESGGGLVQPGGSLRLSCAASGFTFSSYGMYWVRQAPGKGLEWVAKIEQDGSEEYYVDSVKGRFTISRDNAKKSLYLQMNSLRAEDTAVYYCAKGEILPLYFDYWGQGTLVTVSSLEGGGSHHHHHH

SEQ ID NO: 416 - protein, 131 aa, Artificial Sequence
  clone
EVQLVESGGGLVQPGGSLRLSCAASGFTFSSYRMYWVRQAPGKGLEWVASIEQDGSEEYYVDSVKGRFTISRDNAKKSLFLQMNSLRAEDTAVYYCAKGEILPLYFDYWGQGTLVTVSSLEGGGSHHHHHH

SEQ ID NO: 417 - protein, 131 aa, Artificial Sequence
  clone
EVQLVESGGGLVQPGGSLRLSCAASGFTFSSYSMYWVRQAPGKGLEWVAEIKQDGSVQYYVDSVKGRFTISRDNAKNSLYLQMNSLRAEDTAVYYCAKGEILPLYFDYWGQGTLVTVSSLEGGGSHHHHHH

SEQ ID NO: 418 - protein, 138 aa, Artificial Sequence
  clone
QVQLVQSGAEVKKPGASVKVSCKASGYNADAYYINWVRQAPGQGLEWMGSIKPNTGATKYAQKFQGRVTITRDTSISTAYMELSRLRSDDTAVYYCASLDRDTWYPHSYAGWFDAWGQGTLVTVSSLEGGGSHHHHHH

SEQ ID NO: 419 - protein, 131 aa, Artificial Sequence
  clone
EVQLVESGGGLVQPGGSLRLSCAASGFTFSSYSMYWVRQAPGKGLEWVANIKQDGSEKYYVDSVKGRFTISRDNAKNSLFLQMNSLRAEDTAVYYCAKGEILPLHFDYWGQGTLVTVSSLEGGGSHHHHHH

SEQ ID NO: 420 - protein, 131 aa, Artificial Sequence
  clone
EVQLVESGGGLVQPGGSLRLSCAASGFTFSSYSMYWVRQAPGKGLEWVAEIKQDGSEQYYVDSVKGRFTISRDNAKNSLYLQMNGLRAEDTAVYYCAKGEILPLYFDYWGQGTLVTVSSLEGGGSHHHHHH

SEQ ID NO: 421 - protein, 131 aa, Artificial Sequence
  clone
EVQLVESGGGLVQPGGSLRLSCAASGFTFSSYGMYWVRQAPGKGLEWVAKIEQDGSEEYYADSVKGRFTISRDNAKKSLYLQMNSLRAEDTAVYYCAKGEILPLYFDYWGQGTLVTVSSLEGGGSHHHHHH

SEQ ID NO: 422 - protein, 131 aa, Artificial Sequence
  clone
EVQLVESGGGLVQPGGSLRLSCATSGFTFSSYGMYWVRQAPGKGLEWVAEIKQDGSEKYYVDSVKGRFTISRDNAKNSLYLQMNSLRAEDTAVYYCAKGEILPLYFDYWGQGTLVTVSSLEGGGSHHHHHH

SEQ ID NO: 423 - protein, 131 aa, Artificial Sequence
  clone
EVQLVESGGGLVQPGGSLRLSCAASGFTFSSYSMYWVRQAPGKGLEWVAEIKPTGSVQYYVSDVKGRFTISRDNAKNSLYLQMNSLRAEDTAVYYCAKGEILPLYFDYWGQGTLVTVSSLEGGGSHHHHHH

SEQ ID NO: 424 - protein, 131 aa, Artificial Sequence
  clone
EVQLVESGGGLVQPGGSLRLSCAASGFTFSSYSMYWVRQAPGKGLEWVAEIKQDGSVQYYVGGVKGRFTISRDNAKNSLYLQMNSLRAEDTAVYYCAKGEILPLYFDYWGQGTLVTVSSLEGGGSHHHHHH

SEQ ID NO: 425 - protein, 131 aa, Artificial Sequence
  clone
EVQLVESGGGLVLPGGSLRLSCAASGFTFSSYSMYWVRQAPGKGLEWVAEIKQDGSEQYYVDSVKGRFTISRDNAKNSLYLQMNSLRAEDTAVYYCAKGEILPLYFDYWGQGTLVTVSSLEGGGSHHHHHH

SEQ ID NO: 426 - DNA, 15 bp, Artificial Sequence
  linker sequence
ggggsggggsggggs

SEQ ID NO: 427 - DNA, 12 bp, Artificial Sequence
  linker sequence
aaggggsggggs

SEQ ID NO: 428 - DNA, 22 bp, Artificial Sequence
  linker sequence
aaggggsggggsggggsggggs

SEQ ID NO: 429 - DNA, 33 bp, Artificial Sequence
  linker sequence
aaggggsggggsggggsgggggsggggsggggs

SEQ ID NO: 430 - protein, 253 aa, Artificial Sequence
  1.10-3(G4S)-1.1(E1/6Q)
EVQLVESGGGLVQPGGSLRLSCAASGFTFSSYRMYWVRQAPGKGLEWVASIEQDGSEEYYVDSVKGRFTISRDNAKKSLFLQMNSLRAEDTAVYYCAKGEILPLYFDYWGQGTLVTVSSGGGGSGGGGSGGGGSQVQLVQSGGGLVQPGGSLRLSCAASGFTFSSYSMYWVRQAPGKGLEWVANIKQDGSEKYYVDSVKGRFTISRDNAKNSLFLQMNSLRAEDTAVYYCAKGEILPLHFDYWGQGTLVTVSS

SEQ ID NO: 431 - DNA, 759 bp, Artificial Sequence
  clone
gaggtgcagctggtggagtctgggggaggcttggtccagcctggggggtccctgagactctcctgtgcagcctctggattcacctttagtagttatcgcatgtactgggtccgccaggctccagggaaggggctggagtgggtggccagcatagaacaagatggaagtgaggaatactatgtggactctgtgaagggccgattcaccatctccagagacaacgccaagaagtcactgtttctgcaaatgaatagcctgagagccgaggacacggctgtgtattactgtgcgaaaggggaaatactacccctctactttgactactggggccagggaaccctggtcaccgtctcctcaggtggaggaggtagtggtggaggaggtagtggtggaggaggtagtcaggtgcagctggtgcagtctgggggaggcttggtccagcctggggggtccctgagactctcctgtgcagcctctggattcacctttagtagttattcgatgtactgggtccgccaggctccagggaaggggctggagtgggtggccaacataaagcaagatggaagtgagaaatactatgtggactctgtgaagggccgattcaccatctccagagacaacgccaagaactcactgtttctgcaaatgaatagcctgagagccgaggacacggctgtgtattactgtgcgaaaggggaaatactacccctccactttgactactggggccagggaaccctggtcaccgtctcttca

SEQ ID NO: 432 - protein, 267 aa, Artificial Sequence
  3.2-4(G4S)-1.2
QVQLVQSGAEVKKPGASVKVSCKASGYNADAYYINWVRQAPGQGLEWMGSIKPNTGATKYAQKFQGRVTITRDTSISTAYMELSRLRSDDTAVYYCASLDRDTWYPHSYAGWFDAWGQGTLVTVSSAAGGGGSGGGGSGGGGSGGGGSEVQLVESGGGLVQPGGSLRLSCAASGFTFSSYSMYWVRQAPGKGLEWVAEIKQDGSVQYYVSDVKGRFTISRDNAKNSLYLQMNSLRAEDTAVYYCAKGEILPLYFDYWGQGTLVTVSS

SEQ ID NO: 433 - DNA, 771 bp, Artificial Sequence
  clone
caggttcagctggtgcagtctggagctgaggtaaagaagcctggggcctcggtgaaggtctcctgtaaggcttccggatataacgcggacgcctattatataaattgggtgcgacaggcccctggacaaggtcttgagtggatgggaagtatcaagcctaataccggtgccacaaaatatgcacagaagtttcagggcagagtcaccataaccagggacacgtccatcagcacagcctacatggagctgagcaggctgagatctgacgacacggccgtgtattactgtgcgagtctggatcgggatacgtggtacccgcactcctacgcggggtggttcgacgcgtggggccagggaaccctggtcaccgtctcttcagcggccggtggtggcggttcaggtggaggtggtagtgaggttcagttggtggaaagcggcggtggcctggtccagccgggtggtagcctgcgcctgtcctgcgcggctagcggtttcacgtttagcagctacagcatgtactgggtgcgtcaagcgccaggcaaaggtctggaatgggttgccgagattaagcaagacggttctgttcagtattatgtcagcgacgtgaagggtcgttttaccatcagccgtgacaacgcgaaaaacagcctgtatttgcagatgaattccctgcgcgctgaagataccgcggtgtattactgtgcgaaaggtgagattctgccgctgtacttcgattactggggccaaggcaccctggttactgtctcgagc

SEQ ID NO: 434 - protein, 267 aa, Artificial Sequence; identical to SEQ ID NO: 432
  clone

SEQ ID NO: 435 - DNA, 801 bp, Artificial Sequence
  clone
caggttcagctggtgcagtctggagctgaggtaaagaagcctggggcctcggtgaaggtctcctgtaaggcttccggatataacgcggacgcctattatataaattgggtgcgacaggcccctggacaaggtcttgagtggatgggaagtatcaagcctaataccggtgccacaaaatatgcacagaagtttcagggcagagtcaccataaccagggacacgtccatcagcacagcctacatggagctgagcaggctgagatctgacgacacggccgtgtattactgtgcgagtctggatcgggatacgtggtacccgcactcctacgcggggtggttcgacgcgtggggccagggaaccctggtcaccgtctcttcagcggccggtggtggcggttcaggaggtggaggttcaggaggtggtggttctggtggaggtggtagtgaggttcagttggtggaaagcggcggtggcctggtccagccgggtggtagcctgcgcctgtcctgcgcggctagcggtttcacgtttagcagctacagcatgtactgggtgcgtcaagcgccaggcaaaggtctggaatgggttgccgagattaagcaagacggttctgttcagtattatgtcagcgacgtgaagggtcgttttaccatcagccgtgacaacgcgaaaaacagcctgtatttgcagatgaattccctgcgcgctgaagataccgcggtgtattactgtgcgaaaggtgagattctgccgctgtacttcgattactggggccaaggcaccctggttactgtctcgagc

SEQ ID NO: 436 - protein, 277 aa, Artificial Sequence
  clone
QVQLVQSGAEVKKPGASVKVSCKASGYNADAYYINWVRQAPGQGLEWMGSIKPNTGATKYAQKFQGRVTITRDTSISTAYMELSRLRSDDTAVYYCASLDRDTWYPHSYAGWFDAWGQGTLVTVSSAAGGGGSGGGGSGGGGSGGGGSGGGGSGGGGSEVQLVESGGGLVQPGGSLRLSCAASGFTFSSYSMYWVRQAPGKGLEWVAEIKQDGSVQYYVSDVKGRFTISRDNAKNSLYLQMNSLRAEDTAVYYCAKGEILPLYFDYWGQGTLVTVSS

SEQ ID NO: 437 - DNA, 831 bp, Artificial Sequence
  clone
caggttcagctggtgcagtctggagctgaggtaaagaagcctggggcctcggtgaaggtctcctgtaaggcttccggatataacgcggacgcctattatataaattgggtgcgacaggcccctggacaaggtcttgagtggatgggaagtatcaagcctaataccggtgccacaaaatatgcacagaagtttcagggcagagtcaccataaccagggacacgtccatcagcacagcctacatggagctgagcaggctgagatctgacgacacggccgtgtattactgtgcgagtctggatcgggatacgtggtacccgcactcctacgcggggtggttcgacgcgtggggccagggaaccctggtcaccgtctcttcagcggccggtggtggcggttcaggcggaggtggctctggaggtggaggttcaggaggtggtggttctggcggcggtggatcgggtggaggtggtagtgaggttcagttggtggaaagcggcggtggcctggtccagccgggtggtagcctgcgcctgtcctgcgcggctagcggtttcacgtttagcagctacagcatgtactgggtgcgtcaagcgccaggcaaaggtctggaatgggttgccgagattaagcaagacggttctgttcagtattatgtcagcgacgtgaagggtcgttttaccatcagccgtgacaacgcgaaaaacagcctgtatttgcagatgaattccctgcgcgctgaagataccgcggtgtattactgtgcgaaaggtgagattctgccgctgtacttcgattactggggccaaggcaccctggttactgtctcgagc

SEQ ID NO: 438 - protein, 5 aa, Artificial Sequence
  clone
SYGMY

SEQ ID NO: 439 - protein, 17 aa, Artificial Sequence
  clone
KIEQDGSEEYYVDSVKG

SEQ ID NO: 440 - protein, 10 aa, Artificial Sequence
  clone
GEILPLYFDY

SEQ ID NO: 441 - protein, 119 aa, Artificial Sequence
  clone
EVQLVESGGGLVQPGGSLRLSCAASGFTFSSYGMYWVRQAPGKGLEWVAKIEQDGSEEYYVDSVKGRFTISRDNAKNSLYLQMNSLRAEDTAVYYCAKGEILPLYFDYWGQGTLVTVSS

SEQ ID NO: 442 - protein, 5 aa, Artificial Sequence
  clone
SYGMY

SEQ ID NO: 443 - protein, 17 aa, Artificial Sequence
  clone
KIEQDGSVEYYVDSVKG

SEQ ID NO: 444 - protein, 10 aa, Artificial Sequence
  clone
GEILPLYFDY

SEQ ID NO: 445 - protein, 119 aa, Artificial Sequence
  clone
EVQLVESGGGLVQPGGSLRLSCAASGFTFSSYGMYWVRQAPGKGLEWVAKIEQDGSVEYYVDSVKGRFTISRDNAKNSLYLQMNSLRAEDTAVYYCAKGEILPLYFDYWGQGTLVTVSS

SEQ ID NO: 446 - protein, 5 aa, Artificial Sequence
  clone
SYQMY

SEQ ID NO: 447 - protein, 17 aa, Artificial Sequence
  clone
GIKQDGSEQYYVDSVKG

SEQ ID NO: 448 - protein, 10 aa, Artificial Sequence
  clone
GEILPLYFDH

SEQ ID NO: 449 - protein, 119 aa, Artificial Sequence
  clone
EVQLVESGGGLVQPGGSLRLSCAASGFTFSSYQMYWVRQAPGKGLEWVAGIKQDGSEQYYVDSVKGRFTISRDNAKKSLYLQMNSLRAEDTAVYYCAKGEILPLYFDHWGQGTLVTVSS

SEQ ID NO: 450 - protein, 5 aa, Artificial Sequence
  clone
SYGMY

SEQ ID NO: 451 - protein, 17 aa, Artificial Sequence
  clone
EIKQDGSEEYYVDSVKG

SEQ ID NO: 452 - protein, 10 aa, Artificial Sequence
  clone
GEILPLYFDY

SEQ ID NO: 453 - protein, 119 aa, Artificial Sequence
  clone
EVQLVESGGGLVQPGGSLRLSCAASGFTFSSYGMYWVRQAPGKGLEWVAEIKQDGSEEYYVDSVKGRFTISRDNAKNSLFLQMNSLRAEDTAVYYCAKGEILPLYFDYWGQGTLVTVSS

SEQ ID NO: 454 - protein, 5 aa, Artificial Sequence
  clone
SYSMY

SEQ ID NO: 455 - protein, 17 aa, Artificial Sequence
  clone
GIEQDGSEEYYVDSVKG

SEQ ID NO: 456 - protein, 10 aa, Artificial Sequence
  clone
GEILPLYFDY

SEQ ID NO: 457 - protein, 119 aa, Artificial Sequence
  clone
EVQLVESGGGLVQPGGSLRLSCAASGFTFSSYSMYWVRQAPGKGLEWVAGIEQDGSEEYYVDSVKGRFTISRDNAKNSLFLQMNSLRAEDTAVYYCAKGEILPLYFDYWGQGTLVTVSS

SEQ ID NO: 458 - protein, 5 aa, Artificial Sequence
  clone
SYRMY

SEQ ID NO: 459 - protein, 17 aa, Artificial Sequence
  clone
EIEQDGSEQYYVDSVKG

SEQ ID NO: 460 - protein, 10 aa, Artificial Sequence
  clone
GEILPLYFDY

SEQ ID NO: 461 - protein, 119 aa, Artificial Sequence
  clone
EVQLVESGGGMVQPGGSLRLSCAASGFTFSSYRMYWVRQAPGKGLEWVAEIEQDGSEQYYVDSVKGRFTISRDNAKNSLFLQMNSLRAEDTAVYYCAKGEILPLYFDYWGQGTLVTVSS

SEQ ID NO: 462 - protein, 5 aa, Artificial Sequence
  clone
SYGMY

SEQ ID NO: 463 - protein, 17 aa, Artificial Sequence
  clone
EINQDGSEQYYVDSVKG

SEQ ID NO: 464 - protein, 10 aa, Artificial Sequence
  clone
GEILPLYFDY

SEQ ID NO: 465 - protein, 155 aa, Homo sapiens
MTPGKTSLVSLLLLLSLEAIVKAGITIPRNPGCPNSEDKNFPRTVMVNLNIHNRNTNTNPKRSSDYYNRSTSPWNLHRNEDPERYPSVIWEAKCRHLGCINADGNVDYHMNSVPIQQEILVLRREPPHCPNSFRLEKILVSVGCTCVTPIVHHVA

SEQ ID NO: 466 - protein, 119 aa, Artificial Sequence
  clone
EVQLVESGGGLVQPGGSLRLSCAASGFTFSSYGMYWVRQAPGKGLEWVAEINQDGSEQYYVDSVKGRFTISRDNAKNSLYLQMNSLRAEDTAVYYCAKGEILPLYFDYWGQGTLVTVSS